European Patent Application EP 4 365 294 A1, published May 8, 2024. Title: Application of Plant JAZ Protein and its Derived Polypeptides in the Prevention and Treatment of Tumors in Human and Animals. Applicant: Anyang Institution of Sino-cotton Industry Innovation. The sequence listing filed with the application follows.

SEQUENCE LISTING (99 sequences)

SEQ ID NO: 1 - protein, 209 aa, Artificial sequence
  Synthesized
MSRATVELDFFGMEKANSCKSQFQKFLDRRRSFRGIQGAISKMNPELIKSVIASGSTTRNPVDWRKSFSVPSSPKEDRSTSLPSLPLLNPALRSIPSEESPETAPLTIFYNGTVSVINVPRDKVRGSIFKLAVEGSSKNIESVDSSKAANPSSDQQNLLEARNGDLPIARRKSLQRFLEKRKERLDILLCWIRIYRIFTNFLKKKKNNN

SEQ ID NO: 2 - protein, 363 aa, Artificial sequence
  Synthesized
MERDFLGLNSNEPLAVVKDDVNTDKYKQIGFTKSSGIQWPFSNKVFAVPQLMNFNFAQGDKTKKTGYDSKVSPLFMPISTMDASELQKSFNHNWNGGGHFSLTDSHVQHNTNMFPASNQTISVSGSNPFVKNHFTTTGQNFPANTIKPQFLGGVPVTTPHSVLPTLGTVGGSVEPCAQTSGSPAQLTIFYAGEVNVFDDITPEKAQAIMFLAGNGSSMASNSAYPKPPVQTPILKPVQVDSVPANQLINTQLSFGMPSPLPVSSHAGMQSWSGSTSTEEQIICKASVPPTPSTPISKLESPNLVNTMGSDAATGMMPSVPQARKASLARFLEKRKGRIMSTASPYNLISKKSLDYATTMESNA

SEQ ID NO: 3 - protein, 197 aa, Artificial sequence
  Synthesized
MSRASVELDFFGMEKQNFCKSRFQKSLDRRLSFRGLQGALSKVNPELIKTVIASSLKNPQGQDNVYQMDSNKSFSVPSSPKETQSLFPALPLLNPAARATSENGPEIAPLTIFYNGTVSVFNVPRDKAESILKLAVEVEGNSKNVEPIDSKVASPPSDRQQLLETLNGDLPIARRKSLQRFLEKRKERMTCASPYAC

SEQ ID NO: 4 - protein, 240 aa, Artificial sequence
MSSCSESTAMKPARSPEKPSFAQTCNLLSQYLKEKGSFGDLSLGMTCNVEANGTPVVPPPTMNLFPLNDKSDDVCGRNGGNPKNLTSMDLFPQQAGLASKDDSPNKLEPQTAPMTIFYGGQVIVFNDFPANKAKEIMLLASNSSSQSNNSFNPIPFTSSIARSPIESSIGVPPTSKPVHPAQRAVPGDLPIARRASLHRFLEKRKDRITAKAPYQINNSAAAPSLSGDNKSWLGLAAQSP

SEQ ID NO: 5 - protein, 216 aa, Artificial sequence
  Synthesized
MEGEAGSYEDVKPNVVVKQSNGDVVGDNGVGNLGSVDAPDFLSKKNFQNCPAPSQLTIFYDGHVCVFDAIPVEKVREIMLIAATAAAGAANSVDMKKVATDCATTSPVLTRSPSLQSTATATALASPQAQVYPINRTPFCKLKELPIARRHSLQRFFEKRRDRLVNRNPYPNPSTPKSFDDTKANLSAATSPESGCFGKSPVAQEEFHPKAPAHVA

SEQ ID NO: 6 - protein, 226 aa, Artificial sequence
  Synthesized
MTKNFLPNMENSYESLKPNLGASTSKSNAKRCGFFPEIRSFGVSSSKEDTNRMTDFRKPAKVEPKNSQMTIFFGSQVAVFNDFPADKFKEIMDLLPSHGCSTASGGVVDTVMEKVKSKIVQIEPSNHEIPDLNVATATGNSPPPPHDSSVEWHQYGGSGSSDLRIARRNSLHKFFEKRKERATARAPYQVNNARGSTPPPKPNENKSSHEEGQSSKEASRDLDLKL

SEQ ID NO: 7 - protein, 119 aa, Artificial sequence
  Synthesized
MRRNCNLELRLLPSSYPSDSHDMMEERIESPKTQQQQLTIFYNGRVCVSDVTELQAKAILMLANRERDERMKSPTGWEPVSPTLKSQVKCPNTALSMKRSLQRFLQKRKTRIQATSPYH

SEQ ID NO: 8 - protein, 364 aa, Artificial sequence
  Synthesized
MERDFLGLNSKQSFPLVKEEVEEIGFTKSLGIQWPISNKVSSAVPPQQMSFDFAQVDNAKRIGYDSIVSPAFMHISPPDAAQLQKSFNHNRQRVGNHFPFTAASVQHDAHHVQRPYDMKMFPVSNQSVPVSTTNPFMNNHFTTTAMKSQLLGGIPVTSPPHSVLPTLSSFGGSIEPRKSVRGLGDSRSPVQLTIFYAGTVNVYDDITPEKAQAIMLLAGNGSSLTSNVAHPKVQVQAPISKPLQFENLPTNHFTNEQLCSGIPSPLSVSSHTGVQSRSGSTSTDEKTVCKTTGSLTTPISLVESPKLANTMGPVTPTSIMPTVPQARKASLARFLEKRKERIMTASPYDLSKKPPHCTTQGSNA

SEQ ID NO: 9 - protein, 263 aa, Artificial sequence
  Synthesized
MNMSCSPEFLVQKPTRSPEKTSFTQTCNLLSQYLKEKGSFGDLSLGMTCNDEANETPEMLRPTMNLFPVNEKSGDDCLAAPPPRKLRSMDLFPNQAAFSSPKDDALKSTMNKLGSSVEPQTAQMTIFYGGQVIVFNDFPADKAKEIMLLAGKGSSQSNSFNTNPPHINAPFTSTIATSPIESGIGVPPTPNFSTTVTQECIRSAQRSIPGDLPIARRASLHRFLEKRKDRMTTRAPYEISNSTASSSKPGDDKSWLGLAAQSP

SEQ ID NO: 10 - protein, 228 aa, Artificial sequence
  Synthesized
MEEEAESREEVKPNVVVKETNGDIVGDNDAGKLGTIETPDFLSQKIFHNCSLPILASGVITTSPAQSQLTIFYGGKVSVFDAISAEKIQEIMLIAATVAAADVGSVDMKNAATDYATISPALTRCPSLQSTATASASPQAQLYPLPRTSFSKLQAELPIARRHSLQRFLEKRRDRLVNKNPYPGPSTPKMADDVKADVSATTSPESGYFKASPIRQEDIQPKAPAHVA

SEQ ID NO: 11 - protein, 297 aa, Artificial sequence
  Synthesized
MSTGEMVSRSPLYKPLNQLTEDDISQVTREDCRLYLKEKGMRRPSWNKSQAIQQVISLKTLLETTSDSEAVEASKKLHVPFPQNPPRFVSDSTVQPNETTRHKGISVPVNESVPRIRSDPSEFKFSRENSVQTAVSANDSVSPRSASVAKEPSGQMTIFYCGKVNVYDNIPGCKAEAILQFAASPVSFPQETLVDQRTSPLSIPCHVQAAGDKVSQRSPGVILSSMQAVKVAENCRFPRDDCNVSYEDSLEGPTSRNALLQRYLEKKKDRYIRSMMLDQHSAIIAHVDMDGAGVPTE

SEQ ID NO: 12 - protein, 252 aa, Artificial sequence
  Synthesized
MFGSPEYTCLKPASLPEKPLFKRTCSLLSQYLKEKCSFGDLTLGITCNNNVEKGMPEIVRPATETTTTTMDLFPRDHVSGVMRNSRSMDLFPQGAGFSADNGSRRVGVDLETENAAAPMTIFYCGQVIVFNDFPADKAKEIMALASKCSSENPKTNTFVPGSPNESGLGVHSNSNDQVPNIRTNVSTSRECVRSIPGDLPIARRASLHRFLEKRKDRITSKAPYPINGSAGASPPKPGNSKPWLGLAVESLQ

SEQ ID NO: 13 - protein, 125 aa, Artificial sequence
  Synthesized
MRRNCNLELELFPSRMFPGHRQNMVEESKRSPQNQQQQLTIFYNGRVCVCDITELQARAILMRANQETDERIKTPTGSEPDSPTSSSSTSLSRLCSPNAGLSMKKSLQRFLQKRKNRIQATSPYH

SEQ ID NO: 14 - protein, 120 aa, Artificial sequence
  Synthesized
MRRNCNLELRLHPSSYSGGDRVEESSENPENQQQQLTIFYNGRVCVCDVTEIQARAILMIANRETDERLRTPRQGSEPASPMVHSQINSPNNGLSTSMKRSLQRFLQKRKNRIQATSPYH

SEQ ID NO: 15 - protein, 270 aa, Artificial sequence
  Synthesized
MSNLGQKSPDRASFVNLLSQYLKEKRNLGDFSLGMTSKPDAKGLETSRQQAKNMNFLSNMPNCSESSRPNLVASTSNVKSSDFFPEIGSFCASSSKEDTINKTDFMKSAAVEPKNAQLTIFFGGQVLVYNDFPADKVKEIMAVANRGWSTACSGVVADSSMEKLNANLDKIDYSSPHIPDLNITSATVNSSAQDPSVERHQYVGSDLRIARRNSLHKFFEKRKDRAAMRAPYQLINHQGSPPPPKPDENKPSHEEGQSSKETPRDIDLNL

SEQ ID NO: 16 - protein, 337 aa, Artificial sequence
  Synthesized
MSPGETVSRSPLDKPLNQLTEDDISQVTREDCRRYLKEKGMRRPSWNKSQAIQQVISLKTLLETTSDSDAVEARKKLYPPCPEYPPRVVSDSNVLPKEITPNNGILVPVPESVPCPHSNPSKSDFSGDNSGRTVISGNDSVSPRIAGAPKESAGQMTIFYCGKVNVYDDMPGCKAEAILQLAASPVSFPHEILADQRTTPWSIPCHSQAASVKTTPCSQMVILPPQQTENCQFPREESNASLEDSLEGPTRRKASVQRYLEKKKDRFKNKRKLAMSSSPTLDIYLNQVGDQFSNEQLKQSEPYYSPQAEVQRMPLECSSIENVAKIPRLTTDGKGDQ

SEQ ID NO: 17 - protein, 370 aa, Artificial sequence
  Synthesized
MERDFIGLRSKNAAITIKVEPSNAQPDDSVLLRGSGMQLSFSNKVSTVPQFLSFDGARDDKPRKATHDTLLSSGFMTIPAADSNKKPHPGLTQKQGGNHYAATTYGLQQLDGHQSRLSHEARIFPSSSQPNHTITVSMNTPLLQPHLASPGQNIIGHTINPQPFTGVPIMAAPVSVVPPSSPIIGTTDLRNAAKSSRAPAQLTIFYAGSVCVYDDVSPDKAQAIMLLAGNVSSTTQSKTAPVTQPQTHIPRPCTLSPFSGLPNHLSVTSHVSLQPVAGSSGTNELTAATRIGALASTNNQPDPPKLVNPAVAVPQARKASLARFLEKRKERVSNTSPYNICKRSESGPLASDGISFSVTSAGSSPLQAIN

SEQ ID NO: 18 - protein, 206 aa, Artificial sequence
  Synthesized
MSRATVELDFFGMEKANSCKSQFQKFLDRRRSFRGIQGAISKMNPELIKSVIASGSTNRNPVDWRKSFSVPSSPKEDRSTSLPSLPLLNPALRSTPSEDSPETAPLTIFYNGTVSVINVPRDKAESIFKLAVEGSSKNIESVDSSKAANPSSDQQNLLEARNGDLPIARRKSLQRFLEKRKERLDILLCWRRIYRIFTNFLKKNNN

SEQ ID NO: 19 - protein, 362 aa, Artificial sequence
  Synthesized
MERDFLGLNSNEPLAVVKDDVNTDKYKEIGFTKSSGIQWPFSNKVFAVPQLMNFNFAQGDKTKKTGYDSKVSPLFMPISTMDAAELQKSFNHKWNGGNHFSLTDSHVQHNTNMFPASNQTISVSGSDPFVKNHYTTTGQKFPANTIKPQFFGGVPVTTPHSVLPTLGSVGGSVEPCTKASGSPAQLTIFYAGEVNVFDDITPEKAQAIMFLAGNGSSMASNSAYPKPPVQTPILKPVQVDSVPANQLINTQLSFGKPSPLPVSSHAGTQSWSGSTSTEEQIICKASVPSTPSTPISKLESPNLVNTMGSDAATGMMPSVPQARKASLARFLEKRKGRIMSTASPYNLSKKSLDYATTMESNA

SEQ ID NO: 20 - protein, 140 aa, Artificial sequence
  Synthesized
MSHNIDLFRKYLLSKSENHTVGKTNKEESAVMKHRSSPPLTPLIMPPKFASSISRPLSLLERRLLQPTRYLQKSSTTQLTIFYAGVVNVYDNVPTDKAQAIMLLAGESCLTKPTAKEKTLVEAKASPNQQQAVGNNFDRH

SEQ ID NO: 21 - protein, 194 aa, Artificial sequence
  Synthesized
MSRASVELDFFGMEEQICCKSRFQKSLDRRLSFRGLQGALSKVNPELIKSVIASGLKNPQGQDNVYQMDSNKSFSVPSSPKETQSLFPALPLLTPAARATSENGPETAPLTIFYNGTVSVFNVPRDKAESILKLAVEVEGNSKNVEPIDSKVASPPSDRQQLLETLNGDLPIARRKSLQRFLEKRKERYFLFCF

SEQ ID NO: 22 - protein, 240 aa, Artificial sequence
  Synthesized
MSSCSESTAMKPARSLEKPSFAQTCNLLSQYLKEKGSFGGLSLGMTCNVEANGTPVVPPPTMNLFPVNDKSDNVCGRNGGNPKNLASMDLFPQQAGLASKDDSPNKLEPQTAPMTIFYGGRVIVFNDFPANKAKEIMLLASNSSSQSNDSFNPIPFTSSIARSPIKSSIGVPPTSKPVHPAQRAVPGDLPIARRASLHRFLEKRKDRITAKAPYQISHSAAAPSLSGDNKSWLGLAAQSP

SEQ ID NO: 23 - protein, 226 aa, Artificial sequence
  Synthesized
MEGEAGSYEDVKPNVVAKQSNGDVVGDNGVGNLGSVEAPDFLSKKNFQNCSVATPASGLNSTGPAPSQLTIFYDGHVCVFDAIPVEKVREIMLIAATGAANSVDMKKVATDCATTSPVLTRSPSLQSTATATALASPQAQVYPTNRTPFCKLKELPIARRHSLQRFFEKRRDRLVNRNPYPNPSTPKSFDDTKANLSAATSSESGCFGKSPVAQEEFHPKAPAHVA

SEQ ID NO: 24 - protein, 226 aa, Artificial sequence
  Synthesized
MTKNFLPNMDNSYESLKPNLGASTSKSNAKPCGFFPEIRSFGASSSKEDTNMMTDFRKPAKVEPKNSQMTIFFGGQVAVFNDFPADKFKEIMDLLASHGCSTASGVVVDTVMEKVKSKTVQIEPSNHEIPDLNVSTATGNSPPPPHDSSVEWHQYGGSGPSDLRIARRNSLHKFFEKRKERATARAPYQVNNARGSTLPPKPDENKSSHEEGQSSKEASRDLDLKL

SEQ ID NO: 25 - protein, 365 aa, Artificial sequence
  Synthesized
MERDFLGLNSKQSFPLVKEEVEEIGFTKSLGIQWPISNKVSSAVPPQQMSFDFAQGDNAKRMGYDSIVSSTFMHISPPDAAELQKSFNHNRQRVGNHFPFTAASSVQHDVHHVQRPYDMKMFPVSNQSVPVSTTNPFMNSHFTTTAMKSQLLGGIPVTTPPHSVLPTLGSFGGSIEPRKSVRGLGDSRSPVQLTIFYAGTVNVYDDITPEKAQAIMLLAGNGSSLTSNVAHPNVQVQAPISKPLQFETLPTNHFTNAELCSGIPSPLSVSSHTGVQSRSGSTSTDEKTVCKTTGSLTTPISLVESPKLANTMGPVTPTSMMPSVPQARKASLAWFLEKRKERIMTASPYDLSKKPPHCTTQGSNA

SEQ ID NO: 26 - protein, 119 aa, Artificial sequence
  Synthesized
MRRNCNLELRLLPSSYPSDSHDMMEARIESPETQQQQLTIFYNGRVCVSDVTELQAKAILILANRERDERMKSPTGCEPVSPTLKSQVNSPNTSLSMKRSLQRFLQKRKTRIQATSPYH

SEQ ID NO: 27 - protein, 263 aa, Artificial sequence
  Synthesized
MNMSCSPEFMVQKPARSPEKTSFTQTCNLLSQYLKEKGSFGDLSLGMTCNVEANETPEMLRPTMNLFPVNGKSGDDCHAAPPPRKLRSMDLFPNQAAFSSPKDDALKSTMNKLGSSVEPQTAQMTIFYGGQVIVFNDFPADKAKEIMLLAGKGSSQNNSFNPNPPHINAPFTSTIATSPIESGIGVPPTPNFSTTVTQECIRSAQRPIPGDLPIARRASLHRFLEKRKDRMTTSAPYQISNSTASSSKPGNDKSWLGLAAQSP

SEQ ID NO: 28 - protein, 228 aa, Artificial sequence
  Synthesized
MEEEAESREEVKPNVVVKETNGDIVGDNDAGKLGTIETPDFLSQKISHNCSLPILASGVNTTSLAQSQLTIFYGGKVSVFDAISAEKIQEIMLIAAAVAAADVGSVDMKNAATDYATISPALTRCPSLQSTATALASPQAQLYPFPRTSFSKLQAELPIARRHSLQRFLEKRRDRLVNKNPYPGPSTPKMVDGAKADVSATTSPESGCFKASPIRQEDIQPKAPAHVA

SEQ ID NO: 29 - protein, 223 aa, Artificial sequence
  Synthesized
MFGSPEKPMFKRTCSLLSQYLKEKGSFGDLTLGITCSHNVEKGMPEIVRPATETRTTTMDLFPQGAGFSADNGSRRVGVDVDPQNAAAPMTIFYCGQVIVFNDFPADKAKEIMALASKCSSENPKTNTFVPGSPNESGLGVHSNSNDQVPNIRTNLPTSRECVRPIPGDLPIARRASLHRFLEKRKDRITSKAPYPINGSAGASPPKPGNSKPWLGLAVESLQ

SEQ ID NO: 30 - protein, 125 aa, Artificial sequence
  Synthesized
MRRKCNLELELFPSRIFPGHRQNMVEESKRIPQNQQQQLTIFYNGRVCVCDVTELQARAILMRANREADERIKTPTGSEPDSPTSSSSTSPSRLCSPNAGLSMKKSLQRFLQKRKNRIQATSPYH

SEQ ID NO: 31 - protein, 120 aa, Artificial sequence
  Synthesized
MRRNCNLELRLHPSSYSGGDRVEESSENPENQQQQLTIFYNGRVCVCDVTEIQARAILMIANRETDERLRTPRSGSGPASPTVHSQINSPNNGLSTSMKRSLQRFLQKRKNRIQATSPYH

SEQ ID NO: 32 - protein, 270 aa, Artificial sequence
  Synthesized
MSNLGQKSPDRASFVNLLSQYLKEKRNLGDFSLGMTSKPDAKGLETSRQHAKNMNFLSNMPNCSESSRPNLVASTSNVKSSDFFPEIGSFGASSSKEDTFNKTDFMKSAAVEPKNAQLTIFFGGQVFVYNDFPADKVKEIMAVANRGWSTSCSGVVADSAMEKLNANLDKIDYSSPHIPDLNITSATANSPAQDPSVERCQYVGSDLRIARRNSLHKFFEKRKDRAAMRAPYQLNNHQGSPPPPKPDENKPSHEEGQSSKETPRDIDLNL

SEQ ID NO: 33 - protein, 365 aa, Artificial sequence
  Synthesized
MEAGVTTTATTTASFSSILDKPLSQLTEEDISQLTREDCRKFLKEKGMRRPSWNKSQAIQQVISFKALLESNEDSGAGARRKILVCPPPSHFPPQNAVASNSGESVKEAVFGEEESLYGQKDLSLKAAPVVQMNCQGGDTDDKTLSPSLGSPREYSKLPGRSQCETNELGGQMTIFYCGKINVYDGVPLAKARAIMHLAASPIDFPQGNLCNQNGAFRSFLGHVQEAEDKNDLTSSIALNLNSHIMHTEKMTEYQQQFRGKANISRDSDVDGQVSRKVSLQRYLEKRKDRGRFFKGRKNAGQTLSSSEMYLNHQIRAHYLNGQTNQSRTSSPPQSGVPHAFYSSADNQELVNFSVDLNDEGGQEH

SEQ ID NO: 34 - protein, 337 aa, Artificial sequence
  Synthesized
MSPGETVSRSPLDKPLNQLTEDDISQVTREDCRRYLKEKGMRRPSWNKSQAIQQVISLKTLLETTSDSDAVEARKKLYPPCPEYPPRVVSDSNVLPREMTPNNGILVPVSESVPCPLSNPSKSDFSGDNSGRTVISGNDSVSPRIAGAAKEPAGQMTIFYCGKVNVYDDMPGCKAEAIMQLAASPVSFPHEILADQRSTPWSIPCHSQAASVKTTPCSQMVILPPQQTENCQFPREESNASLEDSLEGPTSRKALVHRYLEKKKDRFKNKRKLAMSSSPTLDIYLNQVGDQFSNEQLKQSEPYYSPQAEAHRMPLECSSIENVAKIPRLTTDGKGNR

SEQ ID NO: 35 - protein, 371 aa, Artificial sequence
  Synthesized
MERDFLGLRSKNAAITIKVEPSDAQPNDSVWLRGSGMQLSFTNKVSTVPQFLSFDGARDDKPRKATHDTLLSSGFMTIPTTDSNKKPHPGLTQKQGGNHYAATTYGLQQLDVHQSRLSHEARIFPSSSQLNHTITVSMNTPLLQPHLASPGQNIIGHTINPQPFTGVPIMAAPVSVVPPSSPIIGTTDLRNAAKSSKAPAQLTIFYAGSVCVYDDVSPDKAQAIMLLAGNGSSATQSKTAPVTQRQTHIPRPCTLSPFSGLPNHLSATSHVSLQPVAGSSGTNELTAATRIGALASANNQPDPPKLVNPAVAVPQARKASLARFLEKRKERVSNTSPYNICKRSPESGPLASDGISFPVTSAGSSPLQAIN

SEQ ID NO: 36 - DNA, 630 bp, Artificial sequence
  Synthesized
atgtccagagctaccgtcgagcttgatttcttcggcatggagaaagccaattcctgcaaatctcagttccagaaattccttgatcgccgccggagcttccgaggtattcaaggcgccatttcgaagatgaatccagagcttatcaaatctgtgattgcttccggttcgacgacccggaatccggttgattggagaaaatccttttcggttccgtcgagtcctaaagaagatcggagtacttcgcttccttctttacctctactcaatcctgctttgaggtctattccttctgaggagagtcctgaaacagctccgttgacgattttttacaacggaacggtttccgtaatcaatgtacctcgagacaaggttcgcggaagcatcttcaaacttgccgttgaaggaagctcaaaaaacattgaatcagtagactcatcaaaagctgcaaatccttcaagtgatcaacaaaacctcctcgaagctcgtaatggagatttgccaattgctagaagaaagtcgctgcaaagatttctggaaaagcgcaaagagaggttagatatattactgtgttggatccgaatttacagaatttttactaattttctaaaaaaaaaaaaaaacaacaactga

SEQ ID NO: 37 - DNA, 1092 bp, Artificial sequence
  Synthesized
atggagagagattttctgggtttgaattcaaatgaaccattggctgtggttaaggatgatgttaacactgataagtacaaacaaataggttttactaaaagctcagggatacaatggcccttttcaaacaaagttttcgctgttccacagctgatgaactttaattttgcccaaggggataaaaccaaaaagactggatatgattcaaaagtatcccctctcttcatgcctatatcaacaatggatgcttctgaacttcagaaatcgttcaatcacaattggaatggtgggggtcatttttcattgactgattctcatgttcaacacaacacgaacatgtttccggcatcaaaccagacaatttctgtttctgggagcaacccgttcgtgaagaatcatttcactaccactggtcaaaactttcctgctaatactataaaaccacaatttcttggaggggttccagtgacaactccacattcagttcttcccacccttggcactgttggtggaagtgttgaaccatgcgcccagacctctggatcacctgctcaattgactatcttttatgcgggtgaagtgaatgtctttgatgatattacccctgagaaggctcaagctatcatgtttttggctgggaacgggtcttccatggcttctaattcagcttatccaaaacccccggtccagacacctattttgaaaccagttcaagttgatagtgttcctgcgaaccagctcataaatacacaactgagctttggtatgccaagccctttacctgtttcatctcatgctggtatgcagtcttggagtggatccaccagtaccgaagaacagataatatgcaaggcctcagtacctccaactccatctacccctattagcaaattggagagtccaaatttggtaaataccatgggatctgatgctgccaccggcatgatgccttctgttccacaggctcgcaaagcttccttggctcggtttttggagaagcgcaaggggaggataatgagtacagcatcaccatacaatcttattagcaagaagtctctagattatgcaactaccatggaatcgaatgcataa

SEQ ID NO: 38 - DNA, 594 bp, Artificial sequence
  Synthesized
atgtcgagagctagcgtcgagcttgatttctttggaatggagaaacagaacttctgcaaatctcggtttcagaaatctctcgatcgccgtctaagctttcgaggtcttcaaggcgccctttcgaaggtgaatcctgagcttattaaaaccgtgattgcctctagtttgaagaacccgcagggtcaggataatgtgtatcagatggactccaacaagtctttttcggtcccttccagtcctaaagaaactcagagtctgtttccagctttacctcttcttaaccctgctgccagggctacatccgagaatggtcctgaaatagctcccttaaccattttctacaacggaacggtttccgtttttaatgtacctcgagataaggcggagagcatcttaaaactcgcggttgaagttgaaggaaactcaaaaaatgttgaaccaatagactcaaaagtggcaagtcctcctagcgatcgacaacagcttcttgaaactctcaatggagatttgccaatcgcccggagaaagtctttgcagagatttctggaaaagcgcaaagagaggatgacttgtgcatctccatatgcttgctag

SEQ ID NO: 39 - DNA, 723 bp, Artificial sequence
  Synthesized
atgtcgtcttgctcggaatctacggctatgaaaccggctaggtcaccggagaagccaagttttgcccaaacttgtaatttgttgagccagtacttgaaggagaaaggtagctttggggatctatctctgggaatgacatgcaacgttgaagctaatgggacaccagtggtgccgcctccgaccatgaatctgttccctctcaatgacaagtccgatgatgtttgtggccgaaacggtgggaatcctaagaacttgacatccatggatttgttcccccaacaagctggtttggcttctaaagatgatagtcccaacaagttggagcctcagactgcaccaatgaccatcttttatggtggacaagtgattgtgttcaatgattttccagcaaacaaagctaaggaaatcatgcttttagctagcaacagcagctcacaaagcaacaacagcttcaaccccatcccttttacttctagcatagccagaagtccaatcgaatcaagcattggagttcctcctacctcaaaaccggttcaccctgctcagcgagctgtccctggcgatctgccaattgcaaggagagcttcactgcatcggttcctagagaagcgaaaggataggatcactgcaaaagcgccataccagataaataactcagctgcagctccttccctgtccggcgataacaagtcatggctcggtttggctgctcaatcaccatag

SEQ ID NO: 40 - DNA, 651 bp, Artificial sequence
  Synthesized
atggaaggggaagctggttcatacgaggacgttaagccaaacgtcgtcgttaaacaaagtaatggcgatgttgtcggggataatggtgttggaaatctgggatccgttgacgcccccgattttctttccaagaaaaatttccagaactgccctgctccatctcaactaaccatcttctatgatggacacgtttgtgtgtttgacgcaattcctgtggaaaaggtgcgggagattatgcttattgccgcaactgctgctgctggtgctgctaactctgttgacatgaagaaagttgcaactgattgtgccaccacctcacctgttcttacgaggtctccttcgcttcaaagtactgctactgcaactgctctggcttcaccacaggcacaggtgtaccctattaacaggacccctttctgcaaactgaaagaactaccaattgcaaggagacactcccttcagcgattttttgagaagcggcgggacaggctggtgaacaggaatccatatcctaatccatcaacaccaaaatcatttgatgacaccaaagctaacctcagtgctgcaacttcaccagaatcgggttgctttggtaaatcgcctgttgctcaagaagaattccatccaaaagctccagctcatgttgcataa

SEQ ID NO: 41 - DNA, 681 bp, Artificial sequence
  Synthesized
atgacgaagaactttttgcccaacatggaaaattcttatgagagtttaaaaccgaatctcggggcatctacatcgaaatcaaatgcgaaacgttgtggttttttcccagagattaggagttttggtgtctccagttccaaggaagataccaacaggatgacagatttcaggaaaccagcaaaagtggaaccaaagaattcccagatgaccatattttttggcagtcaagtggcagtatttaatgacttcccagctgacaagttcaaggaaatcatggacttattacctagccatggatgctcaaccgcaagcggtggtgttgttgatactgtcatggaaaaagttaagtctaaaatagtccaaatcgagcccagcaatcatgaaattccagacctgaatgttgctactgcgactgggaatagtcctcctccccctcatgattcttccgttgagtggcatcaatatggcggttcaggatcttcagatcttcgaattgcaagaagaaattcacttcacaagtttttcgaaaagagaaaagaaagggcaacagcaagagcgccataccaagtaaacaacgcaagaggatcgactccaccacctaaacccaatgaaaacaaatcatctcacgaggaaggtcaatcatcgaaagaagcctcaagagatcttgatctcaagttatag

SEQ ID NO: 42 - DNA, 360 bp, Artificial sequence
  Synthesized
atgagacgaaactgcaacttggaacttcgtcttcttccttctagttatcccagcgacagtcacgacatgatggaagaaagaatcgaaagcccaaaaacccagcagcaacagctaacaattttctacaatggaagagtttgcgtatctgatgttacagagcttcaggcaaaagccattctaatgttagcaaaccgggaaagagatgaaagaatgaaaagtccaacgggatgggaaccggtgtcgccgacgttaaaatctcaggtgaaatgcccaaacacagcgctttccatgaagagatcgcttcaacggttcctccagaaacgaaagacgcgaatccaagctacctctccttaccattaa

SEQ ID NO: 43 - DNA, 1095 bp, Artificial sequence
  Synthesized
atggagagagattttctgggtttgaactcaaaacaatccttccctttggttaaagaagaagttgaagaaattggttttaccaaaagcttggggattcaatggccaatttcaaacaaggtttcttcagctgttccaccacagcagatgagttttgattttgctcaagtagataacgctaaaagaattggatatgattcaatagtatcccctgctttcatgcatatctcaccaccagatgctgctcaacttcagaaatccttcaatcacaacaggcaacgagtaggcaatcatttcccattcacagctgcttctgttcagcatgatgcacatcatgttcaacggccttatgacatgaaaatgtttccggtctcgaaccaatcagttcccgtttcaaccaccaacccatttatgaataatcatttcactactactgctatgaaatcacaattgcttggaggaattccagttacgagtccgccgcattcggttcttcccaccctcagttcctttggtggaagcatcgaaccacggaaaagtgtcaggggccttggggactccagatcacctgttcaattgactatcttttatgctggtaccgtgaatgtttacgatgatatcacccccgagaaggctcaggctatcatgttacttgctgggaatggatcttccttgacttctaatgtggcacatccaaaagtccaagtccaggcaccaatttcaaaaccacttcaattcgaaaatcttcccacgaatcatttcacgaatgaacaactttgttctggtatcccaagccctttatcggtttcatctcacactggtgttcaatccaggagtggatccactagtactgatgaaaagaccgtatgcaagaccacaggaagtctgacaacccctattagcctagtggagtctcctaaattggcaaataccatgggacctgttaccccaaccagcattatgcctactgtgccacaggctcgcaaagcatccttggctcggtttttggagaagcgcaaggagaggattatgactgcatcaccatatgatctaagcaagaaacctccacattgtacaacccagggatcaaatgcatga

SEQ ID NO: 44 - DNA, 792 bp, Artificial sequence
  Synthesized
atgaatatgtcgtgttcaccggaatttttggttcagaaaccgacgaggtcaccggagaagacaagctttacccaaacttgtaacttgttgagtcagtacttgaaggagaaaggtagctttggagatctaagtctgggtatgacatgcaacgatgaagctaatgagactcccgagatgctgcgtcccaccatgaatttgtttcctgtcaatgagaaatccggtgatgattgccttgcggcgcctcctcctcggaaactgagatccatggatttgttccctaatcaagctgctttttcatcacctaaagatgatgctctgaaaagcaccatgaacaaattgggttcttcagtggagcctcaaactgcacagatgaccatcttttatggtggacaagtgattgtgttcaacgatttcccggccgacaaagctaaggagatcatgcttttagctggcaaaggcagctctcaaagcaatagcttcaacaccaatcctccccacatcaatgccccctttacttctaccatagcaacaagtccaattgagtccggtatcggggttcctcctacccctaatttcagcaccacggtaactcaagaatgcatacgatctgctcagcgatccattcccggcgatctaccaattgcaaggagagcttcactccaccggttccttgagaagagaaaggataggatgaccacgagggcaccatacgagataagtaactccacagcatcttcatccaagccaggcgacgacaagtcatggctcggtttggctgctcaatctccgtag

SEQ ID NO: 45 - DNA, 687 bp, Artificial sequence
  Synthesized
atggaagaagaggctgaatcacgcgaggaagtcaagccaaacgtcgtcgttaaagagacaaatggagatattgtcggcgataacgatgcaggaaaattgggtaccattgaaacccctgattttctttcccagaaaatattccataactgttccctaccaattctggcatctggagtaattaccacaagccctgctcaatcccaactcaccatcttctatggcggaaaagtttctgtatttgatgcaatttccgctgaaaagatacaagaaattatgcttattgctgctactgtggctgctgctgatgttggctctgttgacatgaagaatgctgcaaccgattatgccaccatttcacctgctcttacaaggtgtccttcacttcaaagtactgcaactgcctcggcttcgccacaggcacagttgtatcctctccccaggacatcttttagcaaactgcaagctgaactaccaattgcaaggagacactcacttcagcgttttcttgagaagcggcgggacaggctggtgaacaagaacccatatcctggtccatcaacaccaaaaatggctgatgacgtcaaagctgacgtgagtgccacaacttcaccagagtctggctacttcaaggcatcacccattcgtcaagaagatatccaaccaaaagctccagctcatgttgcctaa

SEQ ID NO: 46 - DNA, 894 bp, Artificial sequence
  Synthesized
atgtcaacgggagaaatggtttcccggtcacctctatacaagcctctcaaccagctcaccgaggatgacatttctcaggtcactcgcgaagattgccgcctttacctcaaagaaaaagggatgcggagaccttcgtggaacaaatcgcaggcgattcagcaggtcatctcactgaaaactcttctagaaacgacatcggattctgaagctgtcgaagcttccaagaaacttcacgttcccttcccgcaaaatccgcctcgtttcgtttctgattcaaccgttcaaccgaatgaaacgacacggcataaagggatctcggtcccggtaaacgaatccgttcctcgcatccgttcagatccctcggaattcaaattttctcgcgaaaattccgttcaaaccgccgtctctgctaatgattctgtttctccaagatctgcgagtgtagccaaagagccatcaggacagatgacaattttttattgtgggaaagtgaatgtctatgataatatacctggttgtaaggcggaagcaatcttgcagtttgctgcaagcccagtctcatttccacaggaaactctagttgatcaaaggacctcgccattgtccattccatgccatgtacaggctgcaggtgataaagtaagccaacgttcaccaggggttatattgtcatcaatgcaagcagtgaaggttgcagaaaactgtcgatttcctcgagatgactgcaatgtatcttatgaagacagccttgaaggtcccactagcagaaacgcattgttgcaaagatatcttgagaaaaagaaagacagatatattcgaagtatgatgttggaccagcattcagcgattatagcccatgttgacatggatggcgctggagtgccgacagagtag

SEQ ID NO: 47 - DNA, 759 bp, Artificial sequence
  Synthesized
atgtttggttcaccggaatatacatgtctgaaacctgcaagtttgccggagaaaccactgtttaagcgaacttgtagcttgttaagtcagtacttgaaggaaaaatgtagctttggtgatcttactttgggaatcacatgcaataacaacgttgaaaaagggatgccggagatagtccgtccggcgacggagacgacgacgaccaccatggatttatttccgagggatcatgtttctggtgttatgaggaactcaagatccatggatttgttccctcaaggagccggtttttctgccgataacggttcgagacgggtcggggtcgacttggagactgaaaacgccgcagcgccgatgacgatcttttactgcggacaagtgattgtgttcaatgatttcccagctgataaagctaaggaaatcatggctttagcaagcaagtgcagctccgaaaacccgaaaacgaacacgtttgtacccggtagtccgaacgaatccggcctaggagttcattcgaattccaacgatcaggttcctaatatccgaaccaatgtatcaacaagtcgtgaatgcgttcgttccattcccggcgatctacccattgctcgaagagcttcgcttcatcgattcctcgagaagagaaaggataggatcacttcaaaagcaccatacccaataaacggctccgccggggcatcacctccgaaacccggaaatagcaagccgtggctcggtttagctgttgaatcactacagtag

SEQ ID NO: 48 - DNA, 378 bp, Artificial sequence
  Synthesized
atgagacgaaactgcaacttggaactggagctttttccttcacgtatgtttccaggccatcgtcaaaacatggtggaagagagcaaaagaagcccacaaaatcaacagcagcagctaacaattttctataatggaagagtttgcgtttgtgatattacagagcttcaggcaagagctattttaatgagggcaaatcaagaaacggatgaaagaataaaaactccaacaggatcggaaccggattcaccgacatcgtcatcatcgacatccctgtctcgattatgtagccctaatgctggtctttccatgaagaaatcacttcaaaggttccttcaaaaaagaaagaacagaatccaagctacgtccccttaccattaa

SEQ ID NO: 49 - DNA, 363 bp, Artificial sequence
  Synthesized
atgagacgaaactgcaacttggagcttcgtctccatccttctagttattccggcggcgaccgggtggaagagagcagtgaaaacccagaaaatcaacagcaacagttaacgattttctacaatggaagagtttgtgtttgtgatgttacagagatccaggcaagagccattcttatgattgcaaaccgagaaacggatgaacgactaaggactccgaggcagggatcggaaccggcttcaccgatggtacactctcagataaatagtccgaataatggactttccacaagcatgaagagatcgcttcaacggttcctccaaaaacgaaagaatcgaatccaagctacctctccttaccattaa

SEQ ID NO: 50 - DNA, 813 bp, Artificial sequence
  Synthesized
atgtctaatttagggcaaaaatctcctgacagagcaagttttgtcaatcttctaagccagtacttgaaagaaaaaaggaatcttggggatttcagccttggaatgacttcaaaaccagatgctaaagggcttgaaacatctaggcaacaagcaaaaaacatgaattttttgtccaatatgccgaattgttctgagagttcaagaccaaatcttgtggcgtctacctcaaatgtgaaatcttcagatttctttccagagattggcagtttttgtgcttccagttccaaggaagataccattaacaagacagatttcatgaaatcagcagcagtggaaccaaagaatgctcagctgaccatattttttggtggccaagtgcttgtatataatgattttcccgcggacaaggtgaaggagatcatggccgtagctaaccgtggatggtcaactgcatgtagtggtgttgttgccgactcttccatggaaaaactgaatgctaaccttgacaaaattgactacagcagtcctcatatccctgacttgaacatcacctctgcaaccgtgaatagttcagctcaagatccttcggttgagcgacaccaatatgtcggttcagatttgagaattgcaagaagaaactcacttcacaagttctttgaaaagagaaaagacagggcggccatgagagctccataccaactgatcaaccaccaaggttccccgcctccacctaaacccgacgaaaacaagccatctcacgaggaaggtcaatcatcaaaagaaacaccaagagacattgatctcaacttatag

SEQ ID NO: 51 - DNA, 1014 bp, Artificial sequence
  Synthesized
atgtctccgggagaaacggtctcccggtcacctctagacaagcctcttaaccagcttactgaggatgacatttctcaggtcactcgcgaagattgccgccgttacctcaaagaaaaagggatgcggagaccgtcttggaacaaatcgcaggcgattcagcaggtgatctcgttgaaaactcttctagaaacgacgtctgattccgacgccgttgaagctcggaagaaactttaccctccctgcccggaatatccgcctcgcgtcgtttctgattcaaacgttctaccgaaggaaattacaccgaataacgggatcttggttccagttcccgaatccgttccttgtccccattcaaatccctcgaaatccgatttttccggcgacaattctggccgaacggtcatctctggaaatgattctgtttctccaagaattgcaggcgcaccaaaagagtcagcaggacagatgacaatcttttactgtgggaaagtgaatgtctatgatgatatgcctggttgtaaggctgaagcaatcttgcagcttgctgcaagcccagtctcatttcctcacgaaattctagctgatcaaaggaccacaccatggtccattccatgccattcacaggctgcaagtgtcaaaacaaccccatgctcacaaatggttatattgccacctcagcaaacagaaaactgtcaatttcctcgagaagagagcaatgcatctcttgaagacagccttgaaggacctactcgcagaaaagcatcggtgcaaagatatcttgagaagaagaaagacaggtttaagaacaagagaaagttggcaatgtcttcatctccgaccttagacatctacttaaatcaagtgggagatcagttttcaaatgagcagttgaaacaaagtgaaccatattattctccccaagcagaagtgcaacgcatgcctcttgagtgcagctccattgaaaatgttgcaaagattccccgtcttactactgatggaaaaggtgaccagtaa

SEQ ID NO: 52 - DNA, 1113 bp, Artificial sequence
  Synthesized
atggagagagattttatcggtttgaggtccaaaaatgctgcaattacaatcaaagtagagccttccaatgctcagcctgatgattcagtgttgttgaggggttcagggatgcagttgtctttctcaaacaaggtatctacagttcctcagttcttgtcgtttgatggtgctcgagacgataaaccgagaaaagccacgcatgacactctgttgtcatccggttttatgactattccagctgctgattctaacaagaaaccgcatcctggcttgactcagaaacaagggggaaaccactatgcggctaccacctatggtctccaacaactcgatggacaccaatcccgcctttcccacgaagcaaggatatttccaagttcaagtcagccgaatcacacgattacggtttccatgaacactcctcttctccaaccccatcttgcttcccccggacagaacataatcggtcatactataaacccgcaaccttttaccggagttccaatcatggctgcacctgtatctgttgttcctccatcaagtcctatcatcggtactaccgatcttaggaatgctgccaaatcttctagggcaccagctcaattgactatcttttatgctggatctgtatgtgtgtacgatgatgtatctcccgacaaggcccaagctattatgttacttgctggaaacgtttcttctacgactcaaagtaaaacggcacctgtgactcaaccgcagacacatattccacgaccttgtaccttgtcccctttctcgggtcttccaaatcacctttctgtaacctcccatgtcagtttacagcctgttgcaggatctagtggcaccaatgaactaacagctgcaacaaggataggagctttagcatctactaataaccaaccagatcctccaaaattggttaatcctgcagttgctgtgcctcaggctcgtaaagcatccttggctcgatttttagagaagcgtaaagaaagggtatcaaacacctcaccgtacaacatctgcaaaagatctgaatctggccctcttgcatctgatggcataagtttttccgtgacttctgctggatctagtcctttacaagccatcaattaa

SEQ ID NO: 53 - DNA, 621 bp, Artificial sequence
  Synthesized
atgtccagagctaccgtcgagcttgatttcttcggcatggagaaagccaattcctgcaaatctcagttccagaaattcctcgatcgccgccggagcttccgaggtattcaaggtgccatttcgaagatgaatccggaacttatcaaatctgtgattgcttccggttcgacgaaccggaatccggttgattggagaaaatccttttcggttccgtcgagtcctaaagaagatcggagtacttcgcttccttctttacctctactcaatcctgctttgaggtctactccttctgaggatagtcctgaaacagcaccgttgacgattttttacaacggaacggtttccgtaatcaatgtacctcgagacaaggcggaaagcatcttcaaacttgccgttgaaggaagctcaaaaaacattgaatctgtagactcatcaaaagctgcaaatccttcaagtgatcaacaaaacctcctcgaagctcgtaatggagatttgccaattgctagaagaaagtcgctgcaaagatttctggaaaagcgcaaagagaggttagatatattactgtgttggagacgaatttacagaatttttactaattttctaaaaaaaaacaacaactga

SEQ ID NO: 54 - DNA, 1089 bp, Artificial sequence
  Synthesized
atggagagagattttctgggtttgaattcaaatgaaccattggctgtggttaaggatgatgttaacactgataagtacaaagaaataggttttactaaaagctcagggatacaatggcccttttcaaacaaagttttcgctgttccacagctgatgaactttaattttgcccaaggggataaaaccaaaaagactggatatgattcaaaagtatcccctctcttcatgcctatatcaacaatggatgctgctgaacttcagaaatcgttcaatcacaaatggaatggtgggaatcatttttcattgactgattctcatgttcaacacaacacgaacatgtttccggcatcaaaccagacaatttctgtttctgggagcgacccattcgtgaagaatcattacactaccactggtcaaaaatttcctgctaatactataaaaccacaattttttggaggggttccagtgacaactccacattcagttcttcccacccttggctctgttggtggaagtgttgaaccatgcaccaaggcctctggatcacctgctcaattgactatcttttatgcgggtgaagtgaatgtctttgatgatattacccctgagaaggctcaagctatcatgtttttggctgggaacgggtcttccatggcttctaattcagcttatccaaaacccccggtccagactcctattttgaaaccagttcaagttgatagtgtgcctgcgaaccagctcataaatacacaactgagcttcggtaagccaagccctttacctgtttcatctcatgctggtacgcagtcttggagtgggtccactagtaccgaagaacagataatatgcaaggcctcagtaccttcaactccatctacccctattagcaaattggagagtccaaatttggtgaataccatgggatctgatgctgccaccggcatgatgccttctgttccacaggctcgcaaagcttccttggctcggtttttggagaagcgcaaggggaggataatgagtacagcatcaccatacaatcttagcaagaagtctctagattatgcaactaccatggaatcgaatgcataa

SEQ ID NO: 55 - DNA, 423 bp, Artificial sequence
  Synthesized
atgtctcacaacattgatttgtttagaaaatatcttctcagcaaatctgaaaaccataccgttggtaaaaccaacaaggaagaatcagctgtgatgaagcacaggtcctcaccacctcttactcctttaataatgccacctaagtttgcttccagcatttctcggcccctttctcttctcgaacgacggctccttcaaccaaccaggtatttacaaaaatcttcaacaacacaactcacaattttctacgctggggttgttaacgtgtatgacaatgttcccactgataaggcacaagccatcatgcttctggcgggagagagttgtttgacaaagcctaccgcaaaagaaaagactttagtagaggcaaaagcatcacccaaccaacaacaagccgtgggtaataactttgatagacattaa

SEQ ID NO: 56 - DNA, 585 bp, Artificial sequence
  Synthesized
atgtcgagagctagcgtcgagcttgatttctttggaatggaggaacagatctgctgcaaatctcggtttcagaaatccctcgatcgccgtctaagctttcgaggtcttcaaggcgccctttcgaaggtgaatcctgagcttatcaaatccgtgattgcctctggtttgaagaacccgcagggtcaggataatgtgtatcagatggactccaacaagtctttttcggtcccttccagtcctaaagaaactcagagtctgtttccagctttacctcttcttacccctgctgccagggctacatccgagaatggtcctgaaacagctcccttaaccattttctacaacggaacggtttccgtttttaatgtacctcgagataaggcggagagcatcttaaaactcgcggttgaagttgaaggaaactcaaaaaatgttgaaccaatagactcaaaagtggcaagtcctcctagcgatcgacaacagcttcttgaaactctcaatggagatttgccaatcgcccggaggaagtctttgcagagatttctggaaaagcgcaaagagaggtattttttgttttgtttttaa

SEQ ID NO: 57 - DNA, 723 bp, Artificial sequence
  Synthesized
atgtcgtcttgctcggaatctacggctatgaaaccggctaggtcactggagaagccaagttttgcccaaacttgtaatttgttgagtcagtacttgaaggagaaaggtagctttgggggtttatctctgggaatgacatgcaacgttgaagctaatgggacaccagtggtgccgcctccgaccatgaatctgttccctgtcaatgacaagtccgataatgtttgtggccgaaacggtgggaatcctaagaacttggcatccatggatttgttcccccaacaagctggtttggcttctaaagatgatagtcccaacaagttggagcctcagactgcaccaatgaccatcttttatggtggacgagtgattgtgttcaatgattttccagcaaacaaagctaaggaaatcatgcttttagctagcaacagcagctcacaaagcaacgacagcttcaaccccatcccttttacttctagcatagccagaagtccaatcaaatcaagcatcggagttcctcctacctcaaaaccggttcaccctgctcagcgagccgtccctggcgatctgccaattgcaaggagagcttcactgcatcggttcctagagaagcgaaaggataggatcaccgcaaaagcgccataccagataagtcactccgctgcagctccttccctgtccggcgacaacaagtcatggctcggtttggctgctcaatcaccatag

SEQ ID NO: 58 - DNA, 681 bp, Artificial sequence
  Synthesized
atggaaggggaagctggttcatacgaggacgttaagccaaacgtcgtcgctaaacaaagtaatggcgatgttgtcggggataatggtgttggaaatctgggatccgttgaagcccctgattttctttccaagaaaaatttccagaactgttccgtggcaactcctgcatctggactgaattccactggccctgctccatctcaactaaccatcttctatgatggacacgtttgtgtgtttgatgcaattcctgtggaaaaggtgcgggagattatgcttattgctgcaactggtgctgctaactctgttgacatgaagaaagttgcaactgattgtgccaccacctcacctgttcttacgaggtctccttcgcttcaaagtactgctactgcaactgctctggcttcaccacaggcacaggtgtatcctactaacaggacccctttctgcaaactgaaagaactaccaattgcaaggagacactcccttcagcgattttttgagaagcggcgggacaggctggtgaacaggaatccatatcctaatccatcaacaccaaaatcattcgatgacaccaaagctaacctcagtgctgcaacttcatcagaatcgggttgctttggtaaatcacctgttgctcaagaagaattccatccaaaagctccagctcatgttgcataa

SEQ ID NO: 59 - DNA, 681 bp, Artificial sequence
  Synthesized
atgacgaagaactttttgcccaacatggataattcttatgagagtttaaaaccgaatctcggggcatctacatcgaaatcaaatgcgaaaccttgtggttttttcccagagattaggagttttggtgcctccagttccaaggaagataccaacatgatgacagatttcagaaaaccagcaaaagtggaaccaaagaattcccagatgaccatattttttggtggtcaagtggcagtatttaatgacttcccagctgacaagttcaaggaaatcatggacttattagctagccatggatgctcaaccgcaagcggtgttgttgttgatactgtcatggaaaaagttaagtctaaaacagtccaaatcgagcctagcaatcatgaaattccagacctgaatgtttctaccgcgactgggaatagtcctcctccccctcatgattcttccgttgaatggcatcaatatggcggttcaggaccttcagatcttcgaattgcaagaagaaattcacttcacaagtttttcgaaaagagaaaagaaagggcaacagctagagcgccataccaagttaacaacgcaagaggatcgactctgccacctaaacccgatgaaaacaaatcatctcacgaggaaggtcaatcatcgaaagaagcctcaagagatcttgatctcaagttatag

SEQ ID NO: 60 - DNA, 1098 bp, Artificial sequence
  Synthesized
atggagagagattttctgggtttgaactcaaaacaatccttccctttggttaaagaagaagttgaagaaattggttttaccaaaagcttggggattcaatggccaatttcaaacaaggtttcttcagctgttccaccacagcagatgagttttgattttgctcaaggagataacgctaaaagaatgggatatgattcaatagtatcctctactttcatgcatatctcaccaccagatgctgctgaacttcagaaatccttcaatcacaacaggcaacgagtaggcaatcatttcccattcacagctgcttcttctgttcagcatgatgtacatcatgttcaacggccttatgacatgaaaatgtttccggtctcgaaccaatcagttcccgtttcaactaccaacccatttatgaatagtcatttcactactactgctatgaaatcacaattgcttggaggaattccagttacgactccgccgcattcggttcttcccaccctcggttcctttggtggaagcatcgaaccacggaaaagtgtcaggggccttggggactccagatcacctgttcaattgactatcttttatgctggtaccgtgaatgtttatgatgatatcacccccgagaaggctcaggctatcatgttacttgctgggaatggatcttccttgacttctaatgtggcacatccaaatgtccaagtccaggcaccaatttcaaaaccacttcaattcgaaactcttcccacgaatcatttcacgaatgcagaactttgttctggtatcccaagccctttatctgtttcatctcacactggtgttcaatccaggagtggatccactagtactgatgaaaagaccgtatgcaagaccacaggaagtctgacaacccctattagcctagtggagtctcctaaattggcaaataccatgggacctgttaccccaaccagcatgatgccttctgtgccccaggctcgcaaagcatccttggcttggtttttggagaagcgcaaggaaaggattatgactgcatcaccatatgatctaagcaagaaaccaccacattgtacaacccagggatcaaatgcatga

SEQ ID NO: 61 - DNA, 360 bp, Artificial sequence
  Synthesized
atgagacgaaactgcaacttggaacttcgtcttcttccttctagttatcccagcgacagtcacgacatgatggaagcaagaattgaaagcccagaaacccagcagcaacagctaacaattttctacaatggaagagtttgcgtatctgatgttacagagcttcaggcaaaagccattctaatattagcaaaccgggaaagagatgaaagaatgaaaagtccgacgggatgtgaaccggtgtcgccgacgttaaaatcccaggtgaatagcccaaacacatcactttccatgaagagatcgcttcaacggttcctccagaaacgaaagacgcgaatccaagctacctctccttaccattaa

SEQ ID NO: 62 - DNA, 792 bp, Artificial sequence
  Synthesized
atgaatatgtcgtgttcaccggaatttatggttcagaaaccggcgaggtcaccggagaagacaagttttacccaaacttgtaacttattgagtcagtacttgaaggagaaaggtagctttggagatctaagtctgggtatgacatgcaacgttgaagctaatgagactcccgagatgctgcgtcccaccatgaatttgtttcctgtcaatgggaaatccggtgatgattgccatgcggcgcctcctcctcggaaactgagatccatggatttgttccctaatcaagctgctttttcatcacctaaagatgatgctctgaaaagcaccatgaacaaattgggttcttcagtggagcctcaaactgcacagatgaccatcttttatggtggacaagtgattgtgttcaacgatttcccggccgacaaagctaaggagatcatgcttttagctggcaaaggcagctctcaaaacaatagcttcaaccccaatcctccccacatcaatgccccctttacttctaccatagcaacaagtccgattgagtccggtatcggggttcctcctacccctaatttcagcaccacggtaactcaagaatgcatacgatctgctcagcgacccattcccggcgatctaccaattgcaaggagagcttcactccaccggttccttgagaagagaaaggataggatgaccacaagtgcaccataccagataagtaactccacagcatcttcatccaagccaggcaacgacaagtcatggctcggtttggctgctcaatctccgtag

SEQ ID NO: 63 - DNA, 687 bp, Artificial sequence
  Synthesized
atggaagaagaagctgaatcacgcgaggaagtcaagcctaacgtcgtcgttaaagagactaatggagatattgtcggcgataacgatgcaggaaaattgggtaccattgaaacccctgattttctttcccagaaaatatcccataactgttccctaccgattctggcatctggagtaaataccacaagccttgctcaatcccaactcaccatcttctatggcggaaaagtttctgtatttgatgcaatttccgctgaaaagattcaagaaattatgcttattgctgctgctgtggctgctgctgatgttggctctgttgacatgaagaatgctgcaaccgattatgccaccatttcacctgctcttacaaggtgtccttcacttcaaagtactgcaactgctttggcttcgccacaggcacagttgtatcctttccccaggacatcttttagcaaactgcaagctgaactaccaattgcaaggagacactcacttcagcgttttcttgagaagcggcgggacaggctggtgaacaagaacccatatcctggtccatcaacaccaaaaatggttgatggcgccaaagctgacgtgagtgccacaacttcaccagagtctggctgcttcaaggcatcacccattcgtcaagaagatatccaaccaaaagctccagctcatgttgcgtaa

SEQ ID NO: 64 - DNA, 672 bp, Artificial sequence
  Synthesized
atgtttggttcaccggagaaaccaatgtttaagcgaacttgtagcttgttaagtcagtacttgaaggaaaaaggtagctttggtgatcttactttgggaatcacatgcagtcacaacgttgaaaaagggatgccggagatagtccgtccggcgacggagacgaggacgaccaccatggatttgttccctcaaggagccggtttttctgccgataacggttcgagacgggtcggggtcgatgtggaccctcaaaacgcggcagcgccgatgacgatcttttactgcggacaagtgattgtgttcaatgatttcccagctgataaagctaaggaaatcatggctttagcaagcaagtgcagctccgaaaacccgaaaacgaacacgtttgtacccggtagtccgaacgaatccggcctaggagttcattcgaattccaacgatcaggttcctaatatccgaaccaatttaccaacaagtcgcgaatgcgttcgtcccattcccggcgatctacccattgctcgaagagcttcgcttcaccgattcctcgagaagagaaaggataggatcacttcaaaagcaccatacccaataaacggctccgccggggcatcgccgccgaaacccggaaatagcaagccgtggctcggtttagctgttgaatcactgcagtag

SEQ ID NO: 65 - DNA, 378 bp, Artificial sequence
  Synthesized
atgagacgaaagtgcaacttggaactggagctttttccttcacgtatttttccaggccatcgtcaaaacatggtggaagagagcaaaagaatcccacaaaatcaacagcagcagctaaccattttctataatggaagagtttgcgtttgtgatgttacagagcttcaggcaagagctattttaatgagggcaaatcgagaagcggatgaaagaataaaaactccaacaggatcggaaccggattcaccgacatcgtcatcatcgacatccccgtctcgattatgtagccctaatgctggtctttccatgaagaaatcccttcaaaggttccttcaaaaaagaaagaacagaatccaagctacctccccttaccattaa

SEQ ID NO: 66 - DNA, 363 bp, Artificial sequence
  Synthesized
atgaggcgaaactgcaacttggagcttcgtctccatccttctagttattccggcggcgaccgggtggaagagagcagtgaaaacccagaaaatcaacagcaacagttaacgattttctacaatggaagagtttgtgtttgtgatgttacagagatccaggcaagagccattcttatgattgcaaaccgagaaacggatgaacgattaaggactccgaggtcgggatcgggaccggcttcgccgacggtacactctcagataaatagtccgaataatggactttccacaagcatgaagagatcgcttcaacggttcctccaaaaacgaaagaatcgaatccaagctacctctccttaccattaa

SEQ ID NO: 67 - DNA, 813 bp, Artificial sequence
  Synthesized
atgtctaatttagggcaaaaatctcctgacagagcaagttttgtcaatcttctaagccagtacttgaaagaaaaaaggaatcttggggatttcagccttggaatgacttcaaaaccagatgctaaagggcttgaaacatctaggcaacatgcaaaaaacatgaattttttgtccaatatgccgaattgttctgagagttcaagaccaaatcttgtggcatctacctcaaatgtgaaatcttcagatttctttccagagattggcagttttggtgcctccagttccaaggaagatacctttaacaagacagatttcatgaaatcagcagcagtggaaccaaagaatgctcagctgaccatattttttggtggccaagtgtttgtatataatgattttcccgcggacaaggtgaaggagatcatggccgtagctaaccgtggatggtcaacctcatgtagtggtgttgttgccgactctgccatggaaaaactgaatgctaaccttgacaaaattgactacagcagtcctcatatccctgacttgaacatcacctctgcaaccgctaatagtccagctcaagatccttcggtcgagcgatgccaatatgtcggttcagatttgagaattgcaagaagaaactcacttcacaagttctttgaaaagagaaaagacagggcggccatgagagcaccataccaactgaacaaccaccaaggttccccgcctccacctaagcccgacgaaaacaagccatctcacgaggaaggtcaatcatcaaaagaaacgccaagagacattgatctcaacttatag

SEQ ID NO: 68 - DNA, 1098 bp, Artificial sequence
  Synthesized
atggaggctggggtaacgacgacggcgactacaacagcgtcgttcagttcgatacttgataaacccctcagccaactaaccgaagaagacatttctcaactcactcgcgaagactgtcgcaaattcctcaaagaaaaaggaatgcgtaggccgtcatggaacaaatcgcaggcgatccagcaagtgatttcgttcaaggcgttgttggaaagcaacgaagattccggcgccggagctcgccggaaaatccttgtttgtccaccaccgtcacattttcctccgcaaaatgcggtagcttccaattctggtgagtcagtaaaagaagcagtctttggagaagaagaaagcctgtacggccaaaaagatctttctttgaaagctgctccggtggtgcagatgaattgtcagggcggtgacacggatgacaagactctttcgcctagtttaggctctccacgggagtattcaaaattgcctggcagaagtcaatgtgaaacaaatgagttgggtgggcaaatgacaattttttactgtggaaagatcaatgtgtacgatggtgtaccacttgctaaggcacgagcaatcatgcacctggcagcttctcctattgattttcctcagggcaatctatgtaatcaaaatggcgcctttaggtcctttctgggtcatgtacaagaagccgaagacaaaaacgaccttacttcatctattgctttgaacttgaattctcatatcatgcacactgagaagatgacagaatatcagcagcagtttaggggaaaagcaaacatcagtcgtgattctgatgtagatggacaggtgagcagaaaagtatcattgcagcgatatcttgaaaagcgaaaagacaggggaagattctttaaaggcaggaaaaatgcaggacaaactttgtctagctcggagatgtacctgaaccatcagataagagctcactacttaaatggacaaacaaaccagagcagaacaagttctccaccacagtctggagtgccacatgcattttatagctcagctgacaaccaagagcttgtgaatttttctgtagatctcaatgatgaaggtggtcaagaacactga

SEQ ID NO: 69 - DNA, 1014 bp, Artificial sequence
  Synthesized
atgtctccgggagaaacggtctcccggtcacctctagacaagcctctgaaccagcttactgaggatgacatttctcaggtcactcgtgaagattgccgccgttacctcaaagaaaaagggatgcggagaccgtcttggaacaaatcgcaggcgattcagcaggtgatctcgttgaaaactcttctagaaacgacgtctgattccgacgccgttgaagctcggaagaaactttaccctccctgcccggaatatccgcctcgcgtcgtttctgattcaaacgttctaccgagggaaatgacaccgaataacgggatattggttccagtttccgaatccgttccttgtcccctttcaaatccctcgaaatccgatttttccggcgacaattctggccgaacggtcatctccggaaatgattctgtttctccaagaattgcaggtgcagcaaaagagccagcaggacagatgacaatcttttactgtgggaaagtgaatgtctatgatgatatgcctggttgtaaggctgaagcaatcatgcagcttgctgcaagcccagtctcatttcctcacgaaattctagctgatcaaaggtccacaccatggtccattccatgccattcacaggctgcaagtgtcaaaacaaccccatgttcacaaatggttatattgccacctcagcaaacagaaaactgtcaatttcctcgagaagagagcaatgcatctcttgaagacagccttgaaggacctactagcagaaaagcattggtgcatagatatcttgagaagaagaaagacaggtttaagaacaagagaaagttggcaatgtcttcatctccgaccttagacatctacttaaatcaagtgggagatcagttttcaaatgagcagttgaaacaaagtgaaccatattattctccccaagcagaagcacaccgcatgcctcttgagtgcagctccattgaaaatgttgcaaagattccccgccttactactgatggaaaaggtaaccggtaa

SEQ ID NO: 70 - DNA, 1116 bp, Artificial sequence
  Synthesized
atggagagagattttctcggtttgaggtccaaaaatgctgcaattacaatcaaagtagagccctccgatgctcagcctaatgattcagtttggttgaggggttcagggatgcagttgtctttcacaaacaaggtatctacagttcctcagttcttgtcgttcgatggtgctcgagacgataaaccaagaaaagccacgcatgacacgctgttgtcatccggttttatgactattccaactactgattctaacaagaaaccgcatcctggcttgactcagaaacaagggggaaaccactatgcggctaccacctatggtctccaacaactcgatgtacaccaatcccgcctttcccacgaagcaaggatatttccaagttcaagtcagctgaatcacacgattacggtttctatgaacactcctcttctccaaccccatcttgcttcccccggacagaacataatcggtcatactataaacccgcaaccttttaccggagttccaatcatggctgcacctgtatctgttgttcctccatcaagtcctatcatcggtaccaccgatcttaggaatgctgccaaatcttctaaggcaccagctcagttgactatcttctatgctggatctgtatgtgtgtacgatgatgtatctcccgacaaggcccaagctattatgttacttgctggaaacggttcttctgcaactcaaagtaaaacggcacctgtgactcaaaggcagacacatattccacgaccttgtaccttgtcccctttctcgggtcttccaaatcacctttctgcaacctcccatgtcagtttacagcctgttgcaggatctagtggcaccaatgaactaacagctgcaacaaggataggagctttagcatccgctaataaccaaccagatcctcccaaattggttaatcctgcagttgctgtgcctcaggctcgtaaagcatccttggctcggtttttagagaagcgtaaagaaagggtatcaaacacctcaccgtacaacatctgcaaaagatctcctgaatctggccctcttgcatctgatggcataagttttcctgtgacttctgctggatctagtcctttacaagccatcaattaa

SEQ ID NO: 71 - protein, 646 aa, Artificial sequence
  Synthesized
MTDYRFASTMNLWTDDNASVMEAFMSSDLSALWQPPPQSSASTSTPAVVASSAAAAASGAPDLLKSSVAPQSHPSVALFNQETLQQRLQALIEGAHECWTYAIFWQSSYDYSGSAVLGWGDGYYKGEEDKGKRKLKTSSVVAEQEHRKKVLRELNSLISGSTAPTDDAVDEEVTDTEWFFLVSMTQSFVNGGGLPGQALFNSTPVWVVGSERLASSTCERVRQGQVFGLQTMVCIPSANGVVELGSTELITQSSGLMNKVRVLFNFNNSIEAGYLSMCNNIADEGENDPSSLWISDPNSGVEYKESHNNNQNQQIEKSIQFHDNPSSSSLTENPSSIQQQHSQNFGLNFSDYGFDRSNSVRNGNSSHLFKPESEETLNFGESKRSGNVVEENKKKTSPTSRGSHEDGMLSFSSAVFLPSSGMMKSSGGAGDSDNSDIEASVVKEAECVKPLEPEKKPRKRGRKPANGREEPLNHVEAERQRREKLNQRFYALRAVVPNVSKMDKASLLGDAISYINELSTKVQNADLEKQELQKQLEAMKKELAKKDSCPQNPKTSNHLGNRLIELETEVKVIGWDAMIRIQCKRKNHPAARLMAALKELNLDVQHASVTVVNDLMIQQATVKMGNPFYTQEQLRLALISKIGSEI

SEQ ID NO: 72 - DNA, 1941 bp, Artificial sequence
  Synthesized
atgactgactatcgatttgcgtcgacgatgaatctttggacggacgataacgcatcggttatggaagcttttatgagttctgatctttctgctttatggcagcctccgccgcaatcctctgcatccacttccacaccagctgttgttgcttcttctgctgctgctgctgccagtggtgctcccgaccttttgaagtcctctgtggctccccaatctcacccctccgtcgctcttttcaatcaagaaactctccagcagcggctccaagctcttatcgaaggcgcccacgagtgttggacttacgctattttctggcagtcctcctacgattactctggctccgctgtacttggatggggcgatgggtattacaagggcgaagaagataaggggaaaaggaagttgaaaacttcgtctgtagttgcggagcaagagcatcgtaaaaaagtgcttagagagcttaactctttgatttccggttccacagcccccaccgatgatgctgtcgacgaagaagtcaccgataccgagtggttctttttagtttcgatgacgcagtctttcgtcaacggcggcgggctgccgggacaggctcttttcaattctactccggtttgggttgttgggtcggagcgattagctagttcgacgtgcgagcgagtgaggcaagggcaggtttttggtttgcaaaccatggtctgcataccgtctgcaaacggggtggttgaactgggctcaacagaacttatcacgcaaagctcaggtctgatgaataaggttcgggttttatttaatttcaataacagtattgaagctggttatttgtctatgtgtaataatattgctgatgaaggcgaaaatgatccatcttcgctttggatcagtgatccaaatagcggggtcgaatataaagaaagccataacaataatcaaaaccagcagattgaaaagtcaattcagttccatgacaatccgagttccagtagtttaaccgagaatcccagctccattcaacagcagcacagtcagaactttggcttgaatttctccgattatggttttgataggagtaacagtgtgaggaatgggaattcttctcacctgttcaaaccagaatccgaggagacactgaattttggtgagagtaagaggagtgggaatgtggtggaggagaataagaagaagacatcccccacttccagagggagtcatgaagatgggatgctttccttttcttctgctgtattcttgccttcttctggtatgatgaaatccagtggaggtgctggagattcagataactctgatattgaagcttccgtcgttaaagaagctgaatgtgtcaaacctttggagcctgaaaagaagcctaggaaacgagggagaaagccggctaatggtagagaagagcctctgaatcacgtcgaagccgagcgtcaaagaagggagaagcttaaccagaggttttacgccttgcgtgccgtggtacctaacgtgtccaagatggataaagcatcactcctcggtgatgctatttcgtatattaacgagcttagcacaaaggtacaaaatgcagatttagagaaacaagagttgcagaaacaattagaagcaatgaagaaagagctggcaaagaaagattcatgcccacaaaaccccaagacatcgaaccaccttgggaatagactgatagaattggaaaccgaagtgaaggttatcgggtgggacgcaatgattcgaatccaatgcaagagaaagaaccatccggcagcaaggttaatggctgctttaaaggaattaaatcttgatgtgcagcacgctagtgtgacggtagtgaatgacttgatgatccaacaagccaccgtaaagatggggaacccattttacacacaggagcagctcaggctagctctaatatccaaaatcggaagtgagatatag

SEQ ID NO: 73 - protein, 488 aa, Artificial sequence
  Synthesized
MEDDNGLELSLGLSCGASSAKARGKISSSSDTRTEEGDRGVKIVDNFKNFLQAGNEKQDPSVGSQRSDPIKPLENFFNDLSKGNGEVEATVNLNGRGLWGTNSNRSAEIDEDKRSETGSKRKMLFNEINNPKKLEREAHHTDLHEKSKTSHISLTEDGSTAENEDVAESEVEGSTSRLVSHHDDGSKRFMGVSGSAEVPKEVKLGNLNYGNSFQVQSVNVMNAPFSLPMKDSNSVGIPSSSGHTMPGMMQMMPTGNSERSGTQSVNPGNLPVMFGYLPVQLPLLDKDNPWGMVSHPPQFQASYAGRSPPNADKQSDGLKISQASMHTIARNSSEAAQYDGRTFERVKGEGKQHGVEEGSSTRAEEDVKGSSVNLRANATSDRQTAEALTLDFSAIKPGIAADLKFGGSGSYPNLPWVSTTGTGPHGRTISGVTYRFSANQIKIVCACHGTHMSPEEFVRHASEECTNLDNNNGLATFPGTNPAASSQS

SEQ ID NO: 74 - DNA, 1467 bp, Artificial sequence
  Synthesized
atggaggacgataacgggcttgagcttagcttgggtctatcttgtggtgcttcatctgccaaagccagaggcaagattagtagctcctccgatactaggacagaagaaggtgatagaggtgtcaaaatagtggataactttaaaaactttcttcaagctggaaacgagaaacaagaccccagtgtgggttctcagagaagtgatccaataaaacctttggaaaatttctttaatgatctctccaagggtaacggtgaggtagaagctactgttaacttgaatggtagaggtctttggggtacaaacagtaacaggtctgctgaaatcgatgaagataagcggtccgaaacgggtagtaaacgtaagatgttgtttaatgagataaacaatccaaagaagctcgaaagagaagctcatcacacggatttgcatgaaaagtccaaaacatcacatatctccctaacggaagatggctcaactgctgagaatgaagacgttgcggagtctgaagttgagggttcgacctcaaggctggtttcacaccatgatgatggatccaagcgatttatgggagttagtggttctgctgaggtgcctaaggaggttaagctgggaaacttgaattatggtaactcattccaggttcaatcagtcaatgtcatgaatgcacctttctcattgcctatgaaggattctaactctgtcgggatccctagttcatcaggtcatacaatgcctggcatgatgcaaatgatgcctaccggaaatagtgaacggtctgggacccagtctgtgaatcctggaaacttaccggttatgttcgggtacttgcctgttcaacttccactgttggataaggataatccctggggtatggtctctcaccctccgcaattccaggcttcatatgctggcagaagtccacctaatgcagataagcagagtgatggactgaaaatatcacaagcttccatgcatacaattgcgcgcaattcctctgaggctgcacaatatgatggcaggacattcgaaagagtgaaaggtgaaggtaaacagcatggtgtagaggaaggctcctctactcgggcagaggaagatgtaaaaggaagcagcgtgaatctcagagcaaatgctacatctgatcgacaaactgcagaagccttaactcttgatttttctgccataaaacctggaattgctgcagacctgaaatttggtggatctggttcttatccaaatttaccatgggtttcaaccacaggtactggtccacacggcagaactatttctggtgttacttacagattcagcgcaaatcagataaaaatcgtttgtgcttgccatggtacccacatgtcccccgaagagtttgttcgtcatgccagtgaagagtgcaccaatctagataataacaacggtttggcaacatttccaggtaccaatcctgctgcctctagtcagagctga

SEQ ID NO: 75 - protein, 1135 aa, Artificial sequence
  Synthesized
MSSLSRELVFLILQFLDEEKFKETVHRLEQESGFFFNMKYFEDEVHNGNWDEVEKYLSGFTKVDDNRYSMKIFFEIRKQKYLEALDKHDLSKAVEILVKDLKVFATFNEELFREITQLLTLENFRENEQLSKYGDTKSARAIMLVELKKLIEANPLFRDKLQFPNLRNSRLRTLINQSLNWQHQLCKNPRPNPDIKTLFVDHSCGQPNGARAPSPANNPLLGGLPKAGGFPPLGAHGPFQPTPAPVPAPLAGWMSNPSTVTHPAVSGGAIGLGPSSIPAALKHPRTPPTNPSVDYPSGDSDHVSKRTRPMGISDEVNLPVNVLPVTFPGHGHSQTFNAPDDLPKAVARTLNQGSSPMSMDFHPVQQTLLLVGTNVGDIALWEIGSRERLVLKNFKVWDLSACSMPLQAALVKDPAVSVNRVIWSPDGSLFGVAYSRHIVQIYSYHGGDEVRQHLEIDAHVGGVNDLAFSHPNKQLCVVTCGDDKTIKVWEATNGTKQYTFEGHEASVYSVCPHYKENIQFIFSTAIDGKIKAWLYDNMGSRVDYEAPGRWCTTMAYSADGTRLFSCGTSKDGESFIVEWNESEGAVKRTYQGFRKRSLGVVQFDTTKNRYLAAGDDFSIKFWDMDNVQPLTSVDADGGLPASPRIRFNKDGSLLAVSANDNGIKILANSDGMRLLRTLENLSYDASRTSEAPKPTINPISAAAAAAVATSAGLADRSASVVAIAGMNGDARSLGDVKPRITEESSDKSKIWKLTEISEPSQCRSLRLPENLRVTKISRLIFTNSGNAILALASNAIHLLWKWQRSERNSNGKATASVPPQLWQPSSGILMTNDVADTNPEEAVPCFALSKNDSYVMSASGGKISLFNMMTFKTMATFMPPPPPATFLAFHPQDNNIIAIGMDDSTIQIYNVRVDEVKSKLKGHSKRITGLAFSHVLSVLVSSGADSQLCVWNTDGWEKQRSRFLQVPSGRTPTALSDTRVQFHQDQMHFLVVHETQLAIYETTKLERVKQWVPLESSAPITHATFSCDSQLVYSSFLDATVCVFTAANLRLRCRINPSAYLPASVSSNVHPLVIAAHPSEPNEFALGLSDGGVHVFEPLESENKWGVPPPVENGSSSNMAATPSVGAPGSEQAQR

SEQ ID NO: 76 - DNA, 3408 bp, Artificial sequence
  Synthesized
atgtcgtctctcagtagagagcttgtgttcttgatcttacagtttctagatgaggaaaagtttaaagagactgttcacaggcttgaacaggaatctgggtttttctttaatatgaagtattttgaggatgaggtgcataacggaaactgggatgaggttgagaaatacttgtctggtttcaccaaggtagacgacaatcgatattccatgaaaatctttttcgagataagaaagcagaagtatctcgaggcattggataagcatgatctgtccaaggccgtggagatattagtaaaggatttgaaagtttttgccacatttaatgaggaactttttagggaaatcactcagcttttgacgttggagaatttcagggagaatgaacagttgtcaaaatatggagatacaaagtctgctagagcaatcatgttagttgaactcaagaagcttattgaagcaaatcctttattccgtgacaaattacagttcccaaaccttagaaattcaaggttacgcaccctcattaatcagagcttgaattggcagcatcaactttgtaaaaacccgaggccgaatccagatataaaaactctcttcgtggatcactcttgtggacagccaaatggtgcgcgagcaccatcacctgctaacaatcctcttcttggagggttaccaaaggccgggggctttcctccccttggtgctcatgggccttttcaacctacaccagcgccagttccagcaccccttgctggttggatgtcaaacccttctactgtaactcatccagctgtgtctggtggagctattggtcttggtccttcctcaataccagctgcattgaagcatcctaggactcctccaactaatccttctgtagactacccatctggggactctgatcatgtttccaaaaggacaaggcccatggggatttctgatgaggtaaatcttcctgtcaatgtgctgcctgtaacatttcctggccatggtcacagtcagactttcaatgcacccgatgatctgccaaaggcagttgcaagaactttgaatcagggttcatctcctatgagcatggatttccatcccgttcaacagactctacttctagttggtaccaatgttggagacatagcattgtgggaaattggctctcgggagcggctggttttgaagaactttaaagtttgggatcttagtgcttgttcaatgcctcttcaggctgctctagtcaaagatcctgctgtctctgtaaatcgtgtgatttggagccctgatggttctttatttggagttgcttactcgaggcacattgtgcaaatatattcttatcatggtggcgatgaggttcggcagcatctggagattgatgctcatgttggtggagtaaatgatcttgcattttctcatccaaataagcaactttgtgtagtaacttgcggtgatgacaagacgatcaaggtgtgggaggctaccaatggtacaaaacaatatacctttgaaggtcatgaggcttctgtttattctgtctgccctcactataaagaaaacattcagtttatcttttcaacggctatagatggaaagataaaagcatggttatatgataatatgggatcacgtgttgactatgaagctcctggccgttggtgcacaaccatggcctacagtgctgatggtacaaggcttttttcctgtggcaccagtaaagatggggagtcatttatcgtagaatggaatgaaagtgaaggggccgtgaagaggacctatcaaggattccgcaaacgttctttaggtgttgtgcaatttgacaccactaagaataggtatttagctgccggtgatgatttctctatcaaattctgggatatggacaatgttcaacccttgacaagtgttgatgctgatggaggccttccagcaagtccacgcattcgctttaacaaggatggctctctcttggctgtttccgccaatgataatgggattaagattttggcgaattcagatggtatgcgattattgcgcacgttggagaatctttcttatgatgcctcaagaacatcggaagccccaaagcctacaataaatccaatctcagctgctgctgccgcagcggttgctactagtgctggacttgcagacagaagtgcctctgtagttgctattgctggaatgaatggggatgccaggagcttgggggatgtgaaacccagaataacagaagaatcgagtgataaatcaaagatttggaagctaactgaaatcagtgaaccatctcagtgtcgatccttgaggcttcctgaaaacttgagggtgaccaagatatcaaggttaatcttcactaattcaggtaatgctattttggcattggcatcaaatgctattcacttgctctggaagtggcagcgaagtgaacgtaattcaaatggcaaggcaaccgcgagtgtaccacctcagttgtggcaaccatcaagtggcattcttatgacaaatgatgttgctgatacaaatcctgaagaggctgtaccctgttttgctttatccaagaatgattcttatgtaatgtctgcatctggaggaaagatttccttgtttaatatgatgacattcaagacaatggcgactttcatgccaccaccaccaccagcgacttttcttgcattccaccctcaagataacaatattattgctataggcatggacgattcaacgattcagatatataatgttcgtgtggatgaggtgaagagtaagcttaaaggccactccaaaagaataactggccttgccttctctcatgtactgagtgtgcttgtctcatcaggagcagattctcagctttgtgtatggaacactgatggatgggaaaagcagaggtctagattcttgcaggttccatctgggagaacaccaacggcactgtcagacacacgtgtacaattccatcaagaccagatgcattttcttgttgtacatgagactcagcttgccatatatgaaacaacaaagctagaacgtgtgaagcagtgggttccgctcgaatcttctgctccaattactcatgcgacattctcatgtgatagccaactggtgtattccagctttttggatgcaactgtttgtgtctttactgctgcaaacctcagactacgttgccgtataaatccttctgcttatcttcctgctagtgtcagttccaatgttcatccacttgtaattgctgcacatccatctgagccaaatgaatttgcattgggactctcagatggtggggttcatgtctttgagccccttgaatctgaaaacaaatggggtgtgcctccaccagttgaaaacgggtcatccagcaatatggcagcaacaccttcggtcggagctccaggatcagaacaagcacaacgatga

SEQ ID NO: 77 - protein, 471 aa, Artificial sequence
  Synthesized
MEDSAGGASLRSGPDGKKRRVTYFYEPTIGDYYYGQGHPMKPHRIRMAHNLIVHYSLHRRMEINRPFPAGPDDIRRFHTEEYVDFLNAVTPDSISDPAYSRHLKRFNVGEDCPVFDGLFGFCQASAGGSIGAAVKLNRGDADIAINWAGGLHHAKKSEASGFCYVNDIVLGILELLKYHRRVLYVDIDVHHGDGVEEAFYTTDRVMTVSFHKFGDFFPGTGHIRDVGVGNGKYYALNIPLNDGMDDESFRGLFRPIIQKVMEVYQPDAVVLQCGADSLSGDRLGCFNLSVKGHADCLRFLRSFNVPLMVLGGGGYTIRNVARCWCYETAVAVGVEPDNKLPYNEYYEYFGPDYTLHVEVGSMENLNAPRDMEKIRNMLLEQLSRLSHAPSVPFQTTPSTIQPPEEAEEDMDERPKPRIWNGDDYESDPEEDEKPLRRFSNSDVIQLTTDADMRQVSQDLKEVKAEEQPPAP

SEQ ID NO: 78 - DNA, 1416 bp, Artificial sequence
  Synthesized
atggaagactctgctggaggcgcatcattacggtcgggtcccgacgggaagaagcggcgtgtgacatacttctacgagccaacgatcggcgactactattacggtcagggtcacccgatgaaaccccaccggattcgtatggcacacaatctcatcgtccattattctctccaccgtcggatggagattaaccgtcctttccccgccggtcccgacgacatccgtcgctttcacaccgaagagtatgtggacttcctcaacgccgtcacccccgattccatctccgaccccgcttattctcgccatttgaagcgtttcaatgtcggagaggattgccccgtgttcgatgggctttttggtttctgccaggcctccgctggtggctccattggtgccgccgttaagttgaatagaggggatgccgacatcgccatcaattgggctggtggattgcatcatgctaagaaaagcgaggcttctgggttttgctatgttaatgatatcgtgcttgggattcttgagctcctgaaatatcacaggcgtgtgctgtatgtagatattgatgttcatcacggtgatggtgtagaagaggcattttacaccactgacagagttatgactgtgtctttccataaatttggggatttcttcccagggactggacacatcagggatgttggggtgggtaatggcaaatactatgccttgaatattcccttgaatgatgggatggatgatgagagttttcggggtctatttcgtcctatcatccaaaaggtcatggaagtgtatcaaccagatgcagttgttcttcaatgtggagcagattcattgtctggtgacagattgggttgcttcaacttgtctgtgaagggccatgctgattgtcttcgctttcttagatctttcaatgttcccctaatggtcttgggtggaggagggtatactatccgcaatgttgccagatgttggtgctatgagacagctgttgcagttggggttgagcctgataataagctgccttataatgaatattatgagtattttggtccagattatacacttcatgttgaagtgggcagcatggagaacctgaatgcacctagagatatggagaagataaggaacatgctattagagcagctttctagattatctcatgcacccagtgtaccttttcaaacaacaccatccaccatccaaccgcccgaggaggccgaggaggacatggatgaaagaccaaaacctcgcatatggaatggggatgattatgagtctgatcctgaagaggatgagaaacctttacgcagattctccaattctgatgtaatacaacttacaacagatgctgatatgaggcaggtatcacaagatttgaaagaagtgaaagcagaagaacaaccaccggcaccttga

SEQ ID NO: 79 - protein, 589 aa, Artificial sequence
  Synthesized
MEENGNKLHKTMTSQPGMSDVVLGCVMPYIDDPKDRDAVSLVCRRWYELDALTRKHITIALCYTTSPDRLRRRFRHLESLKLKGKPRAAMFNLIPEDWGGYVTPWVNEIAENFNCLKAVHFRRMIVKDSDLEVLARSRGKVLQVLKLDKCSGFSTDGLLHVGRLCRQLRTLFLEESSIIEKDGQWLHELAVNNSVLTNLNFYMTDLVKVSFEDLEFIAQNCRNLASVKISDCEILDLVGFFHAASVLEEFCGGSFNEQPERYTAVSFPPRLCRLGLTYMGKNEMPIVFPFASLLKKLDLLYALLDTEDHCLLIQRCPNLEVLETRNVIGDRGLEVLARSCKRLKRLRIERGADEQEMEDEEGVVSQRGLMALAQGCLELEYLAVYVSDITNASLQYIGTYSKNLCDFRLVLLDREERITDLPLDDGVRDLLRGCEKLRRFALYLRPGGLTDVGLGYIGQYSSKVRWMLLGYVGESDSGLLEFSKGCPSLQKLEMRGCCFSERALAASVMQLTSLRYLWVQGYRASESGHDLLAMARPFWNIELIPRIVGEDPVIEHPAHILAYYSLAGPRTDFPESVIPLDPSAAGISS

SEQ ID NO: 80 - DNA, 1770 bp, Artificial sequence
  Synthesized
atggaggaaaatggtaataagttgcacaaaacgatgacgtcacaacccggtatgtccgatgtcgtattaggctgcgtgatgccgtacatcgacgacccgaaagaccgcgacgccgtatctctagtttgcaggcggtggtacgagctcgacgcgctgactcgtaagcacataacgatcgcgctttgttacacgacgagtcccgatcggttgaggcgacggttccgtcacttggaatccttgaaattgaaagggaagcctcgggctgcgatgtttaatttgatacctgaagattggggtgggtacgttacgccgtgggtgaatgaaatagcggagaatttcaattgcttgaaagccgtccatttcagaagaatgattgttaaagattcggatctggaagttttggctaggtctagagggaaggttttgcaggttttgaagcttgataaatgctctggtttttctactgatggtctcttgcacgttggccgtttgtgccggcaattaagaaccttgttcttggaagagagctcaattattgagaaagatggtcaatggcttcatgagcttgcagtaaataactcagttctcacgaatttaaacttttacatgacagatcttgtgaaagtgagttttgaagaccttgaattcattgctcaaaattgtcgtaatttggcctctgtgaaaattagcgattgtgaaattttggatcttgtcggtttctttcatgctgcttctgttttagaagaattttgtggtggttcgttcaatgagcaaccagaaaggtatactgctgtatcatttcctccgaggttatgccgtttgggtttaacatacatggggaaaaatgaaatgcccattgtgtttccttttgcatcattgcttaaaaagttggatctcctttatgcattgttggacacagaagaccactgcttgttaatccaaagatgccccaacttagaagttcttgagactaggaatgttataggagatagaggattagaagttctcgctcgaagttgtaagagactaaagaggcttagaatcgagcgaggtgctgatgagcaagaaatggaggatgaagaaggtgttgtttcgcaaagaggattaatggctttagctcaaggatgtcttgaattggaatacttggctgtttatgtatctgacatcaccaatgcatcattacaatatattgggacatactcgaaaaatctgtgtgattttcgtctggttttgcttgatcgagaagaaaggataacagatttgcctcttgacgatggagtccgtgatctattgaggggctgtgaaaagcttagaagatttgctctgtatcttcgacctggtggtttaaccgatgtgggacttggttatattggacaatatagttcgaaagtaagatggatgcttctgggatatgttggggaatctgattcggggcttttggagttctccaagggatgccctagcttgcagaaactagaaatgaggggttgttgtttcagtgaacgtgcacttgcagcttccgtgatgcaattaacttctttgaggtacttgtgggtgcaaggatatagagcatcagaatcaggtcatgatctgttagctatggctcgtccattttggaatattgagctaattccccgaatagttggagaggatcctgtgattgagcatccggctcatatactggcatattactccctagctggaccaagaacagatttccctgaaagtgtcattcctttggatccatctgctgctggaatatcaagctaa

SEQ ID NO: 81 - protein, 490 aa, Artificial sequence
  Synthesized
MHHHHHHENLYFQGMSSCSESTAMKPARSPEKPSFAQTCNLLSQYLKEKGSFGDLSLGMTCNVEANGTPVVPPPTMNLFPLNDKSDDVCGRNGGNPKNLTSMDLFPQQAGLASKDDSPNKLEPQTAPMTIFYGGQVIVFNDFPANKAKEIMLLASNSSSQSNNSFNPIPFTSSIARSPIESSIGVPPTSKPVHPAQRAVPGDLPIARRASLHRFLEKRKDRITAKAPYQINNSAAAPSLSGDNKSWLGLAAQSPMVSKGEEDNMAIIKEFMRFKVHMEGSVNGHEFEIEGEGEGRPYEGTQTAKLKVTKGGPLPFAWDILSPQFMYGSKAYVKHPADIPDYLKLSFPEGFKWERVMNFEDGGVVTVTQDSSLQDGEFIYKVKLRGTNFPSDGPVMQKKTMGWEASSERMYPEDGALKGEIKQRLKLKDGGHYDAEVKTTYKAKKPVQLPGAYNVNIKLDITSHNEDYTIVEQYERAEGRHSTGGMDELYK

SEQ ID NO: 82 - DNA, 1470 bp, Artificial sequence
  Synthesized
atgcatcaccaccaccaccacgaaaacctatacttccaaggaatgtcaagctgcagcgagagcaccgcgatgaagccggcgcgtagcccggaaaaaccgagcttcgcgcagacctgcaacctgctgagccaatatctgaaggagaaaggcagctttggtgacctgagcctgggcatgacctgcaacgttgaagcgaacggtaccccggtggtgccgccgccgaccatgaacctgttcccgctgaacgacaagagcgacgatgtgtgcggccgtaacggtggcaacccgaaaaacctgaccagcatggacctgttcccgcagcaagcgggtctggcgagcaaggacgatagcccgaacaaactggagccgcagaccgcgccgatgaccatcttctacggtggccaagtgattgttttcaacgattttccggcgaacaaggcgaaagaaatcatgctgctggcgagcaacagcagcagccaaagcaacaacagcttcaacccgatcccgtttaccagcagcattgcgcgtagcccgatcgagagcagcatcggtgtgccgccgaccagcaaaccggttcacccggcgcaacgtgcggttccgggtgacctgccgattgcgcgtcgtgcgagcctgcaccgttttctggaaaagcgtaaagatcgtatcaccgcgaaagcgccgtaccagattaacaacagcgcggcggcgccgagcctgagcggtgacaacaaaagctggctgggtctggcggcgcaaagcccgatggttagcaaaggcgaggaagataacatggcgatcattaaggagttcatgcgttttaaagtgcacatggaaggcagcgttaacggtcacgagttcgaaatcgagggtgaaggcgagggtcgtccgtacgagggtacccagaccgcgaagctgaaagttaccaagggtggcccgctgccgtttgcgtgggacatcctgagcccgcaatttatgtacggcagcaaggcgtatgtgaaacacccggcggacattccggattatctgaagctgagcttcccggagggttttaaatgggaacgtgttatgaactttgaggatggtggcgtggttaccgtgacccaggacagcagcctgcaagatggcgaattcatctacaaggttaaactgcgtggcaccaactttccgagcgacggtccggtgatgcagaagaaaaccatgggttgggaggcgagcagcgaacgtatgtatccggaggatggcgcgctgaagggtgaaattaaacagcgtctgaagctgaaagacggtggccactacgatgcggaagttaagaccacctataaagcgaagaaaccggttcaactgccgggcgcgtacaacgtgaacatcaagctggacattaccagccacaacgaggattacaccatcgtggaacagtatgagcgtgcggaaggtcgtcacagcaccggtggcatggacgaactgtataaa

SEQ ID NO: 83 - protein, 207 aa, Artificial sequence
  Synthesized
MSSCSESTAMKPARSPEANGTPVVPPPTMNLFPLNDKSDDVCGRNGGNPKNLTSMDLFPQQAGLASKDDSPNKLEPQTAPMTIFYGGQVIVFNDFPANKAKEIMLLASNSSSQSNNSFNPIPFTSSIARSPIESSIGVPPTSKPVHPAQRAVPGDLPIARRASLHRFLEKRKDRITAKAPYQINNSAAAPSLSGDNKSWLGLAAQSP

SEQ ID NO: 84 - DNA, 624 bp, Artificial sequence
  Synthesized
atgtcgtcttgctcggaatctacggctatgaaaccggctaggtcaccggaggctaatgggacaccagtggtgccgcctccgaccatgaatctgttccctctcaatgacaagtccgatgatgtttgtggccgaaacggtgggaatcctaagaacttgacatccatggatttgttcccccaacaagctggtttggcttctaaagatgatagtcccaacaagttggagcctcagactgcaccaatgaccatcttttatggtggacaagtgattgtgttcaatgattttccagcaaacaaagctaaggaaatcatgcttttagctagcaacagcagctcacaaagcaacaacagcttcaaccccatcccttttacttctagcatagccagaagtccaatcgaatcaagcattggagttcctcctacctcaaaaccggttcaccctgctcagcgagctgtccctggcgatctgccaattgcaaggagagcttcactgcatcggttcctagagaagcgaaaggataggatcactgcaaaagcgccataccagataaataactcagctgcagctccttccctgtccggcgataacaagtcatggctcggtttggctgctcaatcaccatag

SEQ ID NO: 85 - protein, 210 aa, Artificial sequence
  Synthesized
MSSCSESTAMKPARSPEKPSFAQTCNLLSQYLKEKGSFGDLSLGMTCNVEANGTPVVPPPTMNLFPLNDKSDDVCGRNGGNPKNLTSMDLFPQQAGLASKDDSPNKLEPQTASSSQSNNSFNPIPFTSSIARSPIESSIGVPPTSKPVHPAQRAVPGDLPIARRASLHRFLEKRKDRITAKAPYQINNSAAAPSLSGDNKSWLGLAAQSP

SEQ ID NO: 86 - DNA, 633 bp, Artificial sequence
  Synthesized
atgtcgtcttgctcggaatctacggctatgaaaccggctaggtcaccggagaagccaagttttgcccaaacttgtaatttgttgagccagtacttgaaggagaaaggtagctttggggatctatctctgggaatgacatgcaacgttgaagctaatgggacaccagtggtgccgcctccgaccatgaatctgttccctctcaatgacaagtccgatgatgtttgtggccgaaacggtgggaatcctaagaacttgacatccatggatttgttcccccaacaagctggtttggcttctaaagatgatagtcccaacaagttggagcctcagactgcaagcagctcacaaagcaacaacagcttcaaccccatcccttttacttctagcatagccagaagtccaatcgaatcaagcattggagttcctcctacctcaaaaccggttcaccctgctcagcgagctgtccctggcgatctgccaattgcaaggagagcttcactgcatcggttcctagagaagcgaaaggataggatcactgcaaaagcgccataccagataaataactcagctgcagctccttccctgtccggcgataacaagtcatggctcggtttggctgctcaatcaccatag

SEQ ID NO: 87 - protein, 211 aa, Artificial sequence
  Synthesized
MSSCSESTAMKPARSPEKPSFAQTCNLLSQYLKEKGSFGDLSLGMTCNVEANGTPVVPPPTMNLFPLNDKSDDVCGRNGGNPKNLTSMDLFPQQAGLASKDDSPNKLEPQTAPMTIFYGGQVIVFNDFPANKAKEIMLLASNSSSQSNNSFNPIPFTSSIARSPIESSIGVPPTSKPVHPAQRAVPGNNSAAAPSLSGDNKSWLGLAAQSP

SEQ ID NO: 88 - DNA, 636 bp, Artificial sequence
  Synthesized
atgtcgtcttgctcggaatctacggctatgaaaccggctaggtcaccggagaagccaagttttgcccaaacttgtaatttgttgagccagtacttgaaggagaaaggtagctttggggatctatctctgggaatgacatgcaacgttgaagctaatgggacaccagtggtgccgcctccgaccatgaatctgttccctctcaatgacaagtccgatgatgtttgtggccgaaacggtgggaatcctaagaacttgacatccatggatttgttcccccaacaagctggtttggcttctaaagatgatagtcccaacaagttggagcctcagactgcaccaatgaccatcttttatggtggacaagtgattgtgttcaatgattttccagcaaacaaagctaaggaaatcatgcttttagctagcaacagcagctcacaaagcaacaacagcttcaaccccatcccttttacttctagcatagccagaagtccaatcgaatcaagcattggagttcctcctacctcaaaaccggttcaccctgctcagcgagctgtccctggcaataactcagctgcagctccttccctgtccggcgataacaagtcatggctcggtttggctgctcaatcaccatag

SEQ ID NO: 89 - protein, 252 aa, Artificial sequence
  Synthesized
MGHPPLLPLLLLLHTCVPASWGLRCMQCKTNGDCRVEECALGQDLCRTTIVRLWEEGEELELVEKSCTHSEKTNRTLSYRTGLKITSLTEVVCGLDLCNQGNSGRAVTYSRSRYLECISCGSSDMSCERGRHQSLQCRSPEEQCLDVVTHWIQEGEEGRPKDDRHLRGCGYLPGCPGSNGFHNNDTFHFLKGDAFSMNHIDVSCCTKSGCNHPDLDVQYRSGAAPQPGPAHLSLTITLLMTARLWGGTLLWT

SEQ ID NO: 90 - DNA, 759 bp, Artificial sequence
  Synthesized
atgggtcacccgccgctgctgccgctgctgctgctgctccacacctgcgtcccagcctcttggggcctgcggtgcatgcagtgtaagaccaacggggattgccgtgtggaagagtgcgccctgggacaggacctctgcaggaccacgatcgtgcgcttgtgggaagaaggagaagagctggagctggtggagaaaagctgtacccactcagagaagaccaacaggaccctgagctatcggactggcttgaagatcaccagccttaccgaggttgtgtgtgggttagacttgtgcaaccagggcaactctggccgggctgtcacctattcccgaagccgttacctcgaatgcatttcctgtggctcatcagacatgagctgtgagaggggccggcaccagagcctgcagtgccgcagccctgaagaacagtgcctggatgtggtgacccactggatccaggaaggtgaagaagggcgtccaaaggatgaccgccacctccgtggctgtggctaccttcccggctgcccgggctccaatggtttccacaacaacgacaccttccacttcctgaaaggtgacgccttcagcatgaaccacattgatgtctcctgctgtactaaaagtggctgtaaccacccagacctggatgtccagtaccgcagtggggctgctcctcagcctggccctgcccatctcagcctcaccatcaccctgctaatgactgccagactgtggggaggcactctcctctggacctaa

SEQ ID NO: 91 - protein, 251 aa, Artificial sequence
  Synthesized
MGHPPLLPLLLLLHTCVPASWGLRCMQCKTNGDCRVEECALGQDLCRTTIVRLWEEGEELELVEKSCTHSEKTNRTLSYRTGLKITSLTEVVGGGSFHNNDTFHFLKCCNTTKCNEGPILELENLPQNGRQCYSCKGNSTHGCSSEETFLIDCRGPMNQCLVATGTHEPKNQSYMVRGCATASMCQHAHLGDAFSMNHIDVSCCTKSGCNHPDLDVQYRSGAAPQPGPAHLSLTITLLMTARLWGGTLLWT

SEQ ID NO: 92 - DNA, 756 bp, Artificial sequence
  Synthesized
atgggtcacccgccgctgctgccgctgctgctgctgctccacacctgcgtcccagcctcttggggcctgcggtgcatgcagtgtaagaccaacggggattgccgtgtggaagagtgcgccctgggacaggacctctgcaggaccacgatcgtgcgcttgtgggaagaaggagaagagctggagctggtggagaaaagctgtacccactcagagaagaccaacaggaccctgagctatcggactggcttgaagatcaccagccttaccgaggttgtgggaggaggatcattccacaacaacgacaccttccacttcctgaaatgctgcaacaccaccaaatgcaacgagggcccaatcctggagcttgaaaatctgccgcagaatggccgccagtgttacagctgcaaggggaacagcacccatggatgctcctctgaagagactttcctcattgactgccgaggccccatgaatcaatgtctggtagccaccggcactcacgaaccgaaaaaccaaagctatatggtaagaggctgtgcaaccgcctcaatgtgccaacatgcccacctgggtgacgccttcagcatgaaccacattgatgtctcctgctgtactaaaagtggctgtaaccacccagacctggatgtccagtaccgcagtggggctgctcctcagcctggccctgcccatctcagcctcaccatcaccctgctaatgactgccagactgtggggaggcactctcctctggacctaa

SEQ ID NO: 93 - protein, 255 aa, Artificial sequence
  Synthesized
MGLKITSLTEVVCGLDLCNQGNSGRAVTYSRSRYLECISCGSSDMSCERGRHQSLQCRSPEEQCLDVVTHWIQEGEEGRPKDDRHLRGCGYLPGCPGSNGFHNNDTFHFLKCCNTTKCNEGPILELENLPQNGRQCYSCKGNSTHGCSSEETFLIDCRGPMNQCLVATGTHEPKNQSYMVRGCATASMCQHAHLGDAFSMNHIDVSCCTKSGCNHPDLDVQYRSGAAPQPGPAHLSLTITLLMTARLWGGTLLWT

SEQ ID NO: 94 - DNA, 768 bp, Artificial sequence
  Synthesized
atgggcttgaagatcaccagccttaccgaggttgtgtgtgggttagacttgtgcaaccagggcaactctggccgggctgtcacctattcccgaagccgttacctcgaatgcatttcctgtggctcatcagacatgagctgtgagaggggccggcaccagagcctgcagtgccgcagccctgaagaacagtgcctggatgtggtgacccactggatccaggaaggtgaagaagggcgtccaaaggatgaccgccacctccgtggctgtggctaccttcccggctgcccgggctccaatggtttccacaacaacgacaccttccacttcctgaaatgctgcaacaccaccaaatgcaacgagggcccaatcctggagcttgaaaatctgccgcagaatggccgccagtgttacagctgcaaggggaacagcacccatggatgctcctctgaagagactttcctcattgactgccgaggccccatgaatcaatgtctggtagccaccggcactcacgaaccgaaaaaccaaagctatatggtaagaggctgtgcaaccgcctcaatgtgccaacatgcccacctgggtgacgccttcagcatgaaccacattgatgtctcctgctgtactaaaagtggctgtaaccacccagacctggatgtccagtaccgcagtggggctgctcctcagcctggccctgcccatctcagcctcaccatcaccctgctaatgactgccagactgtggggaggcactctcctctggacctaa

SEQ ID NO: 95 - protein, 150 aa, Artificial sequence
  Synthesized
MDFFRVVENQQPPATMPLNVSFTNRNYDLDYDSVQPYFYCDEEENFYQQQQQSELQPPAPSEDIWKKFELLPTPPLSPSRRSGLCSPSYVAVTPFSLRGDNDGGGGSFSTADQLEMVTELLGGDMVNQSFICDPDDETFIKNIIIQDCMW

SEQ ID NO: 96 - DNA, 453 bp, Artificial sequence
  Synthesized
atggatttttttcgggtagtggaaaaccagcagcctcccgcgacgatgcccctcaacgttagcttcaccaacaggaactatgacctcgactacgactcggtgcagccgtatttctactgcgacgaggaggagaacttctaccagcagcagcagcagagcgagctgcagcccccggcgcccagcgaggatatctggaagaaattcgagctgctgcccaccccgcccctgtcccctagccgccgctccgggctctgctcgccctcctacgttgcggtcacacccttctcccttcggggagacaacgacggcggtggcgggagcttctccacggccgaccagctggagatggtgaccgagctgctgggaggagacatggtgaaccagagtttcatctgcgacccggacgacgagaccttcatcaaaaacatcatcatccaggactgtatgtggtaa

SEQ ID NO: 97 - protein, 215 aa, Artificial sequence
  Synthesized
MDFFRVVENQQPPATMPLNVSFTNRNYDLDYDSVQPYFYCDEEENFYQQQQQSELQPPAPSEDIWKKFELLPTPPLSPSRRSGLCSPSYVAVTPFSLRGDNDGGGGSFSTADQLEMVTELLGGDMVNQSFICDPDDETFIKNIIIQDCMWSGFSAAAKLVSEKLASYQAARKDSGSPNPARGHSVCSTSSLYLQDLSAAASECIDPSVVFPYPLN

SEQ ID NO: 98 - DNA, 648 bp, Artificial sequence
  Synthesized
atggatttttttcgggtagtggaaaaccagcagcctcccgcgacgatgcccctcaacgttagcttcaccaacaggaactatgacctcgactacgactcggtgcagccgtatttctactgcgacgaggaggagaacttctaccagcagcagcagcagagcgagctgcagcccccggcgcccagcgaggatatctggaagaaattcgagctgctgcccaccccgcccctgtcccctagccgccgctccgggctctgctcgccctcctacgttgcggtcacacccttctcccttcggggagacaacgacggcggtggcgggagcttctccacggccgaccagctggagatggtgaccgagctgctgggaggagacatggtgaaccagagtttcatctgcgacccggacgacgagaccttcatcaaaaacatcatcatccaggactgtatgtggagcggcttctcggccgccgccaagctcgtctcagagaagctggcctcctaccaggctgcgcgcaaagacagcggcagcccgaaccccgcccgcggccacagcgtctgctccacctccagcttgtacctgcaggatctgagcgccgccgcctcagagtgcatcgacccctcggtggtcttcccctaccctctcaactaa

SEQ ID NO: 99 - DNA, 1706 bp, Artificial sequence
  Synthesized
aagcttgcatgcctgcaggtcaacatggtggagcacgacacacttgtctactccaaaaatatcaaagatacagtctcagaagaccaaagggcaattgagacttttcaacaaagggtaatatccggaaacctcctcggattccattgcccagctatctgtcactttattgtgaagatagtggaaaaggaaggtggctcctacaaatgccatcattgcgataaaggaaaggccatcgttgaagatgcctctgccgacagtggtcccaaagatggacccccacccacgaggagcatcgtggaaaaagaagacgttccaaccacgtcttcaaagcaagtggattgatgtgataacatggtggagcacgacacacttgtctactccaaaaatatcaaagatacagtctcagaagaccaaagggcaattgagacttttcaacaaagggtaatatccggaaacctcctcggattccattgcccagctatctgtcactttattgtgaagatagtggaaaaggaaggtggctcctacaaatgccatcattgcgataaaggaaaggccatcgttgaagatgcctctgccgacagtggtcccaaagatggacccccacccacgaggagcatcgtggaaaaagaagacgttccaaccacgtcttcaaagcaagtggattgatgtgatatctccactgacgtaagggatgacgcacaatcccactatccttcgcaagacccttcctctatataaggaagttcatttcatttggagaggacctcgacctcaacacaacatatacaaaacaaacgaatctcaagcaatcaagcattctacttctattgcagcaatttaaatcatttcttttaaagcaaaagcaattttctgaaaattttcaccatttacgaacgatatctagaggatccttaattaacatggtgagcaagggcgaggagctgttcaccggggtggtgcccatcctggtcgagctggacggcgacgtaaacggccacaagttcagcgtgtccggcgagggcgagggcgatgccacctacggcaagctgaccctgaagttcatctgcaccaccggcaagctgcccgtgccctggcccaccctcgtgaccaccttcggctacggcgtgcagtgcttcgcccgctaccccgaccacatgaagcagcacgacttcttcaagtccgccatgcccgaaggctacgtccaggagcgcaccatcttcttcaaggacgacggcaactacaagacccgcgccgaggtgaagttcgagggcgacaccctggtgaaccgcatcgagctgaagggcatcgacttcaaggaggacggcaacatcctggggcacaagctggagtacaactacaacagccacaacgtctatatcatggccgacaagcagaagaacggcatcaaggtgaacttcaagatccgccacaacatcgaggacggcagcgtgcagctcgccgaccactaccagcagaacacccccatcggcgacggccccgtgctgctgcccgacaaccactacctgagctaccagtccgccctgagcaaagaccccaacgagaagcgcgatcacatggtcctgctggagttcgtgaccgccgccgggatcactctcggcatggacgagctgtacaagggtaccggcgcgcctgagcagaaactcatctctgaagaggatctgtagtgagagctcgaatttccc